European Patent Specification EP 3 993 623 B1, published February 19, 2025. Title: TRANSGENIC MAMMALS AND METHODS OF USE THEREOF. Applicant: TRIANNI, INC. The sequence listing filed with the application follows.

SEQUENCE LISTING (295 sequences)

SEQ ID NO: 1 - DNA, 300 bp, Bos taurus
caggtgcagctgcgggagtcgggccccagcctggtgaagccgtcacagaccctctccctcacctgcacggtctctggattctcattgagcgacaaggctgtaggctgggtccgccaggctccagggaaggcgctggagtggctcggtggtatagacactggtggaagcacaggctataacccaggcctgaaatcccggctcagcatcaccaaggacaactccaagagccaagtctctctgtcagtgagcagcgtgacaactgaggactcggccacatactactgtactactgtgcaccag

SEQ ID NO: 2 - DNA, 293 bp, Bos taurus
caggtgcagctgcgggagtcgggccccagcctggtgaagccctcacagaccctctccctcacctgcacggtctctggattctcattgagcagctatggtgtaggctgggtccgccaggctccagggaaggcgctggagtgtcttggtggtataagtagtggtggaagcacaggctataacccagccctgaaataccggctcagcatcaccaaggacaactccaagagccaagtctctctgtcactgagcagcgtgacaactgaggacacggccacatactactgtgcgaagga

SEQ ID NO: 3 - DNA, 293 bp, Bos taurus
caggtgcagctgcgggagtcgggccccagcctggtgaagccctcacagaccctgtccctcacctgcacggtctctggattctcattaagcgataatagtgtaggctgggtccgccaggctccaggaaaggcgctggagtggctcggtgtcatatatagtggtggaagcacaggctataacccagccctgaaatcccggctcagcatcaccaaggacaactccaagagccaagtctctctatcactgagcagcgtgacaactgaggacacggccacatactactgtgcaagaga

SEQ ID NO: 4 - DNA, 293 bp, Bos taurus
caggtgcagctgcgcgagtcgggccccagcctggtgaagccctcacagaccctctccctcacctgcacggtctctggattctcattgagcagctatgctgtaagctgggtccgccaggctccagggaaggctctggagtggcttggtgatataagcagtggtggaagcacaggctataacccagccctgaaatcccggctcagcatcaccaaggacaactccaagagccaagtctctctgtcagtgagcagcgtgacacctgaggacacggccacatactactgtgcgaagga

SEQ ID NO: 5 - DNA, 293 bp, Bos taurus
caggtgcagctgcgggagtcgggccccagcctggtgaagccctcacagaccctctccctcacctgcacggtctctggattctcactgagcagctatgctgtaggctgggtccgccaggctccagggaaggcgctggagtggctcggtggtataagcagtggtggaagcacatactataacccagccctgaaatcccggctcagcatcaccaaggacaactccaagagccaagtctctctgtcagtgagcagcgtgacacctgaggacacggccacatactactgtgcgaagga

SEQ ID NO: 6 - DNA, 293 bp, Bos taurus
caggtgcagctgcgggagtcgggccccagcctggtgaagccctcacagaccctctccctcacctgcacgatctctggattctcattgagcagctatgctgtaggctgggtccgccaggctccggggaaggcgctggagtgggttggtggtataagtagtggtggaagcacatgccttaacccagccctgaaatcccggctcagcatcaccaaggacaactccaagagccaagtctctctgtcagtgagcagcgtgacaactgaggacacggccacatactactgtgcgaagga

SEQ ID NO: 7 - DNA, 293 bp, Bos taurus
caggtgcagctgcaggagtcgggccccagcctggtaaagacctcacagaccctctccctcacctgcacggcctctggattatcattaaccagatatggtatacactgggtccgccaggctccaggaaaggcgctggagtggcttggtgatataagcagtggtggaagcacaggctataacccaggcctgaaatcccggctcagcatcaccaaggacaactccaagagccaagtctctctgtcactgagcagcctgacacctgaggactcagccacatactactgtgcaagaga

SEQ ID NO: 8 - DNA, 293 bp, Bos taurus
caggtgcagctgcgggagtcgggccccagcctggtgaagccctcacagaccctctccctcacctgcacggtctctggattctcattgagcagcaatggtgtaggctgggtccgccaggctccagggaaggcgctggagtgggttggtggtatagataatgatggagacacatactataacccagccctgaaatcccggctcagcatcaccaaggacaactccaagagccaagtctctctgtcagtgagcagcgtgacacctgaggacacggccacatactactgtgcaaaaga

SEQ ID NO: 9 - DNA, 293 bp, Bos taurus
caggtgcagctgcgggagtcgggccccagcctggtgaagccctcacagaccctctccctcacctgcacggtctctggattctcattgagcagcaatggtgtagtctgggtccgccaggctccagggaaggcgctggagtggctcggtggtatatgcagtggtggaagcacaagctttaacccagccctgaaatcccggctcagcatcaccaaggacaactccaagagccaagtctctctgtcagtgagcagcgtgacacctgaggacacggccacatactactgtgcaagaga

SEQ ID NO: 10 - DNA, 293 bp, Bos taurus
caggtgcagctgcaggagtcgggccccagcctggtgaagccctcacagaccctgtccctcacctgcacggtctctggattctcattaagcgacaatgctgtaggctgggtccgccaggctccaggaaaggcgctggagtagcttggtggtatagataatgatggatacacaaggtataacccagccctgaaatcccggctcagcattaccaaggacaactccaagagctaagtctctgtgtcagtgagcagcgtgacaactgaggactcggccgtgtactactgtgcgaagga

SEQ ID NO: 11 - DNA, 293 bp, Bos taurus; identical to SEQ ID NO: 6

SEQ ID NO: 12 - DNA, 293 bp, Bos taurus
caggtgcagctgcaggagtcgggccccagcctggtgaagacctcacagacactctccctcacttgcacggcctctggattatcattaaccagatatggtatacactgggtccgccaggctccaggaaaggcgctggagtggcttggtgatataagcagtggtggaagcacaggctataacccaggcctgaaatcccggctcagcatcaccaaggacaactccaagagccaagtctctctgtcactgagcagcctgacgcctgaggactcagccacatactactgtgcaagaga

SEQ ID NO: 13 - DNA, 293 bp, Bos taurus
aaggtgcagctgcaggagtcgggtcccagcctggtgaagccctcacagaccctctccctcacctgcacgacctctggattctcattgaccagctatggtgtaagctgggtccgccaggctccagggaaggcgctggagtggctcggtggtatagatagtggtggaagcacaggctataacccaggcctgaaatccaggctcagcatcaccagggacaactccaagagccaagtctctctgtcagtgagcagcgtgacacctgaggacacggccacatactactgtgcgaagga

SEQ ID NO: 14 - DNA, 288 bp, Bos taurus
gaggtgcagctgcgggagtggggccccagcctggtgaagccctcacagaccctctccctcaccttcatggtctctggattctcattgaccagctatggtgtagattgggtccgccaggctccagggaaggtgccggaatgggttggtggtataagcagtggtggaagtacatactataacccagccctgaaattcccggctcagcatcacgagggaaacctccaagagccaagtctctctgagcagcgtgacaactgaggacacggccgtgcactactgtgtgaagga

SEQ ID NO: 15 - DNA, 288 bp, Bos taurus
aaggtgcagctgcgggagtggggccccagcctggtgaagccctcacagaccctctccctcaccttcatggtctctggattctcattgaccagctatggtgtagattgggtccgccaggctccagggaaggtgccggaatgggttggtggtataagcagtggtggaagtacatactataacccagccctgaaattcctggctcagcatcacgagggaaacctccaagagccaagtctctctgagcagcgtgacaactgaggacacggccgtgcactactgtgtgaagga

SEQ ID NO: 16 - DNA, 285 bp, Bos taurus
aaggtgcagctgcaggagtcgggtcccagcctggtgaagccctcacagaccctctccctcacctgcacggtctctggattctcattgagcagctatggtatacactgggtccgccaggctccaggaaaggcgctggagtggcttggtgatataagcagtggtggaagcacaggctataacccaggcctgaaatcccggctcagcatcaccaaggacaactccaagagccaagtctctctgtcactgagcagcctgacgcctgaggacacagccacatactactgt

SEQ ID NO: 17 - DNA, 311 bp, Bos taurus
ccgatgcagctgcaggagtcaggccccagcctggtgaagccctcacagaccctttccttcacctgcactgtgtctggattctcattaaccaacaatggtgtaggctgggtccgccaggctccacaaaagggattggagttggttggtatcatatgtacaatatgatatatatatgatatggaagcacatactaccacccagcccttaagtccaggctcagcatcaccagcgacatctccaagagcctagtctcttgtattactgagcagcgtgacaactgaggacacggccctgtagtactgtgcaaaaga

SEQ ID NO: 18 - DNA, 287 bp, Bos taurus
cagatgagctgcagcagtcgggccagaactggtgaaccctcactcaccctctcctgacgtgcactgtctcttcttactccatcacgtggttattgtcggaactggattcgccaggccctagggaaggggctagagcagatgtcataaataagctatgatggtgacacttactacagcccctgcatcaagatcacacctccatctgcagagacatccaagaatcagttctctctgcagctgagctctgtgaccactgaggacacggcagtgtgctgctgtgcaagaga

SEQ ID NO: 19 - DNA, 294 bp, Bos taurus
caggtgaaggtgcaggagtcgggcccagacctggtgaagccctcgcagatcgtctccctcacatgtgctgtctctggttactccatcacgtggttatggtgagagctgggtccaccaggccccagcgaaggggctagagtggatgggaagcatatattataatggtgacacttaccacagcccctccatcaagagccacacctccatctccaggggcacgtctaagaaccagtcctccctgcagctgagctccgtgaccactgtggacacagctgtgtattactgtgcaagaga

SEQ ID NO: 20 - DNA, 155 bp, Bos taurus
ccagtgcagctgcaggagcagggtccagaactgcggaagctctcacctgtgccatctctggttgctccatcaccaatggttactggtaaccagtactccctgcagctaagctctgtgacaaccaaggacacggcagtatgctgctgtgcaagaga

SEQ ID NO: 21 - DNA, 271 bp, Bos taurus
ccagatgcactgcagcagtcgggcccagaactagtgagccctcactgaccctctcctcacgtgcactatctctggttactccatcaagtggttattgagggaactggttttgccaggccccagggaaggggctagagcagatggcatgcataaactaagatggtgacacttactacatcccctccatcaagagccacacctccaatcagttctccctgcagctgaactctgtgaccattgaggacacggccatgtgttgctgggcaagaga

SEQ ID NO: 22 - DNA, 296 bp, Bos taurus
caggtgaaggtgcaggagtcgggcccagagacctggtgaagccctcgcagatcgtctccctcacatgtgctgtctctggttactccatcacgtggttatggtgggagctggatccaccaggccccagcgaaggggctagagtagatgggaagcatatattataatggtgacacttaccacagcccctccttcaagagccacacgtccatctccaggggcacgtctaagaaccagtcctccctgcagctgagctccgtgaccactgtggacacagctgtgtgttactgtgcaagaga

SEQ ID NO: 23 - DNA, 155 bp, Bos taurus
ccagtgcagctgcaggagcagggtccagaactgcggaagctctcacctgtgccatctctggttgctccatcaccagtggttactggtaaccagtactccctgcagctaagctctgtgacaaccaaggacacggcagtatgctgctgtgcaagaga

SEQ ID NO: 24 - DNA, 155 bp, Bos taurus
ccagtgcagctgcaggagcagggtccagaactgcggaagctctcacctgtgccatctctggttgctccatcaccagtggttactggtaaccagtactccctgcagctaagctctgtgatgaccaaggacacggcagtatgctgctgtgcaagaga

SEQ ID NO: 25 - DNA, 291 bp, Bos taurus
cccagatgcactgctgcagtcgggccagaactggtgaagccctcactgactgtctcctcacttgcactgtctctgcttactccatcacgtggttattgtgggaactggattcgccaggccccagggaaggggctagagcagatgacatgcataaactatgatggtgacacttactacagcccctccatcaagagccacatctccatctgcagggacatccaagaatcagttctccctgcagctgagctctgtgaccactgaggacacggccatgtgttgctgtgcaagaga

SEQ ID NO: 26 - DNA, 294 bp, Bos taurus
caggtgaaggtgcaggagtcgggcccagaactggtgaagccctcgcagatcgtctccctcacatgtgctgtctctggttactccatcacgtggttatggtgggagctggatccaccaggcccgagggaaggggctagagtagatgggaagcatatattataatggtgacacttaccacagcccctccatcaagagccacacgtccatctccaggggcacgtctaagaaccagtcctccctgcagctgagctctgtgaccactgaggacacagctgtgtattactgtgcaagaga

SEQ ID NO: 27 - DNA, 155 bp, Bos taurus
ccagtgcagctgcaggagcagggtccagaactgcggaagctctcacctgtgccatctctggttgctccatcaccagtggttactggtaaccagtactccctgcagctaagctctgtgacgaccaaggacacggcagtatactgctgtgcaagaga

SEQ ID NO: 28 - DNA, 155 bp, Bos taurus
ccagtgcagctgcaggagcagggtccagaactgcggaagctctcacctgtgccatctctggttgctccatcaccagtggttactggtaaccagtactccctgcagctaagctctgtgatgaccaaggacacggcagtatactgctgtgcaagaga

SEQ ID NO: 29 - DNA, 292 bp, Bos taurus
caggtgaaggtgcaggagtcgggcccagaactggtgaagccctcgcagatcatctccctcacatgtgctgtctctggttactccatcacgtggttatggtgggagctggatccaccaggccccagggaaggggttagagtggatgggaagcatatattataatggtgacacttaccacagcccctccatcaagagccacacctccatctgcagagacatccaacaatcagttctccctgtagctgagctctgtgaccactgaggacacagctctgtgttgctgtgcaagaga

SEQ ID NO: 30 - DNA, 291 bp, Bos taurus; identical to SEQ ID NO: 25

SEQ ID NO: 31 - DNA, 294 bp, Bos taurus
caggtgaaggtgcaggagtcgggcccagaactggtgaagccctcgcagatcgtctccctcacatgtgctgtctctggttactccatcacgtggttatggtgggagctggatccaccaggccccagggaaggggctagagtggatgggaagcatatattataaaggtgacacttaccacagcccttccatcaagagccacacgtccatctccaggggcacgtctaagaaccagtcctccctgcagctgagctctgtgaccactgaggacacagctgtgtattactgtgcaagaga

SEQ ID NO: 32 - DNA, 171 bp, Bos taurus
ccagtgcagctgcaggagtagggcccagaactgctgaagctctcactgaccctctccctcacctgtgccatctctggttgctccatcaccagtgcttactggtaaccagtactccctgcagctaagctctgtgatgaccaaggacacggcagtgtgttgctgtgcaagaga

SEQ ID NO: 33 - DNA, 288 bp, Bos taurus
caggtgtcctgcagcagttgggcccagaactggtgagccctcagagaccctctcctcacatgtgctatctctgcttacaccatcatgtggttatagtcagaagtggattcgccaggccgcagggaaggggctagagcagatggcatgcataaactatgatggtgacacttactacagcccctccattaagagccacacctccatctcagagacatccaagaatcagttctccctgctactgagctctgtgaccactgaggacatggccgtgtgttgctgtgcaagaga

SEQ ID NO: 34 - DNA, 288 bp, Bos taurus; identical to SEQ ID NO: 33

SEQ ID NO: 35 - DNA, 296 bp, Bos taurus
caggtgcagctgcaggaatcaggcccggaactgataaagtcttcacagacactctccctcacctgtgctggttctggttactccatcaccagtgattatggtaggaactggatccgccaggccccagggaagggtctagagcagatgggatgcatgtattataatggtgacacttattacagcccctccatcaagagtcacacctccatctgcagagacacacccaagaaccagttctccctgcagctgagctctgtgcccacagaggacacagccatgtgttacttggcaagaaa

SEQ ID NO: 36 - DNA, 289 bp, Bos taurus
caggtgcagctggtgcagtgggggctgagctgaggaagcctggggcctcagtgaaggtgtcctgcaaggcttctggatataccttcaccgactacatgcactgggtgtgacaggcccctcagcaagagcttgaacggatggacagattgacagcaaagatggtggagcaaagtacgcacagaagttccagggcagagtcacgttggctgcagacacgtccaccagcatcacctacgtggagctgagcagtctgaggtctgacgacacggctgtttattactgtgtgaga

SEQ ID NO: 37 - DNA, 289 bp, Bos taurus; identical to SEQ ID NO: 36

SEQ ID NO: 38 - DNA, 289 bp, Bos taurus; identical to SEQ ID NO: 36

SEQ ID NO: 39 - DNA, 294 bp, Bos taurus
caggtgcagctggtgctgttggggctgagctgaggaagcctggggcctcagtgaaggtgtcctgcaaggcttctggatacaccttcaccgactactacacgcactaggtgtgacaggcccctcagcaagggcttgaacagatggacagattgacagcaaagatggtggagcaaagtacgcacagaagttccagggcagagtcacgttggctgcagacacgtccaccagcaccgccgacatggagctgagcagtctgaggtctgaggacacggctgtttattactgtgtgagaca

SEQ ID NO: 40 - DNA, 290 bp, Bos taurus
caggtgcagctggtgccgttggggctgagctgaggaagcctggggcctcagtgaaggtgtcctgcaaggcttctggatacaccttcaccgactacatgcactgcgtgtgacaggcccctcagcaagggcttgaacggatggatggactgaccctcaacatggtggaactaggtacacctagaagttccagagcagagtgatcttggttgcacacacgcccaccaacaccgcctacatggagcagagcagtctgagtctgaggacacggctgtttattactgtgtgaggta

SEQ ID NO: 41 - DNA, 291 bp, Bos taurus
cagttgcagctggtgccattggggctgagctgaggaagcctggggcctcagtgaaggtgtcctgcaaggcttctggatacaccttcaccgactacatgcactgggtgtgacaggcccctcaacaagggcttgaaaggatggacagattgacagcaaagatggtggagcaaagtatgcacagaagttccagggcagagtcacgttggctgcagacacgtccaccagcaccgcctacatggagctgagcagtctgaggtctgaggacacggctgtttattactgtgtgagaca

SEQ ID NO: 42 - DNA, 291 bp, Bos taurus
caggtgcagctggtgctgttgtggctgagctgaggaagcctggggcctcagtgaaggtgtcctgcaaggcttctggatacaccttcaccgactacatgcactgggtgtgacaggcccctcagcaagggcttgaagggatggacagattgacagcaaagatggtggagcaaagtatgcacagaagttccagggcagagtcacgttggctgcagacacgtccaccagcactgcctacatggagctgagcagtctgaggtctgaggacatggctgtttattactgtgtgagaca

SEQ ID NO: 43 - DNA, 289 bp, Bos taurus
caggtgcagctggtgcagtgggggctgagctgaggaagcctggggcctcagtgaaggtgtcctgcaaggcttctggatacaccttcaccgactacatgcactgcgtgtgacaggcccctcagcaagggcttgaacggatggatggactgaccctcaacatggtggaactaggtacacctagaagttccagagcagagtgatcttggttgcacacacgtccaccaacaccgcctacatggagcagagcagtctgaggtctgaggacacggctgtttattactgtgtgagg

SEQ ID NO: 44 - DNA, 291 bp, Bos taurus
caggtgcagctggtgccattggggctgagctgaggaagcctggggcctcagtgaaggtgtcctgcaaggcttctggatacaccttcaccgactacatgcactgcatgtgacaggcccctcagcaagggcttgaaaggatggacagattgacagcaaagatggtggagcaaagtatgcacagaagttccagggcagagtcaccttggttgcagacccgtgcacctgcactgcctacatggagctgagcagtctgaggtctgaggacacggctgtttattactgtgtgagaca

SEQ ID NO: 45 - DNA, 290 bp, Bos taurus
caggtgcagctggtgcagtgggggctgagctgaggaagcctggggcctcagtgaaggtgtcctgcaaggcttctggatacaccttcaccgactacatgcactgcgtgtgacaggcccctcagcaagggcttgaacggatggatggactgaccctcaacatggtggaacaaggtacacctagaagttccagagcagagtgatcttggttgcacacacgcccaccaacaccgcctacatggagcagagcagtctgagtctgaggacacggctgtttattactgtgtgaggta

SEQ ID NO: 46 - DNA, 291 bp, Bos taurus; identical to SEQ ID NO: 44

SEQ ID NO: 47 - DNA, 290 bp, Bos taurus
caggtgcagctggtgccgttggggctgagctgaggaagcctggggcctcagtgaaggtgtcttgcaaggcttctggatacaccttcaccgactacatgcactgcatgtgacaggcccctcagcaagggcttgaacggatggatagattgacagcaaagatggtggagcaaagtatgcacagaagttccagggcagagtcacgttgctgcagacacgtccaccagcaccgcctacatggagctgagcagtctgaggtctgaggacacggctgtttattattgtgtgagaca

SEQ ID NO: 48 - DNA, 294 bp, Bos taurus
caggtgcagctggtgcagtgggggctgagctgaggaagcctggggcctcagtgaaggtgtcctgcaaggcttctggatacaccttcaccgactactacacgcactaggtgtgacaggcccctcagcaagggcttgaacagatggacagattgacagcaaagatggtggagcaaagtacgcacagaagttccagggcagagtcacgttggctgcagacacgtccaccagcaccgccgacatggagctgagcagtctgaggtctgaggacacggctgtttattactgtgtgagaca

SEQ ID NO: 49 - DNA, 291 bp, Bos taurus
caggtgcagctggtgcagtgggggctgagctgaggaagcctggggcctcagtgaaggtgtcctgcaaggcttctggatacaccttcaccgactacatgcactgcgtgtgacaggcccctcagcaagggcttgaacagatggacagattgacagcaaagatggtggagcaaagtatgcacagaagttccagggcagagtcacgttggctgcagacacgtccaccagcaccgccgacatggagctgagcagtctgaggtctgaggacacggctgtttattactgtgtgagaca

SEQ ID NO: 50 - DNA, 284 bp, Bos taurus
caggtacagttggggctgagctaaggaagcctggggcctcagtgaaggtgtcctgcaaggcttctggatacaccttcaccaactactacatgcactgggtgtgacaggaccctcagcaatggcttgaatggatggacagattgacagcaaagatggtggagcaaagtatgcacagaagttccagggcagagtcacgttggctgcagacacgtccaccagcaccgcctacatggagctgagcagtctgaggtctgaggacacggctgttattactgtgtgaaaca

SEQ ID NO: 51 - DNA, 31 bp, Bos taurus
agaataccgtgatgatggttactgctacacc

SEQ ID NO: 52 - DNA, 16 bp, Bos taurus
ttactatagtgaccac

SEQ ID NO: 53 - DNA, 36 bp, Bos taurus
gtattgtggtagctattgtggtagttattatggtac

SEQ ID NO: 54 - DNA, 43 bp, Bos taurus
gtagttatagtggttatggttatggttatagttatggttatac

SEQ ID NO: 55 - DNA, 42 bp, Bos taurus
atgatacgataggtgtggttgtagttattgtagtgttgctac

SEQ ID NO: 56 - DNA, 58 bp, Bos taurus
gtagttgttatagtggttatggttatggttgtggttatggttatggttatgattatac

SEQ ID NO: 57 - DNA, 67 bp, Bos taurus
gtagttatggtggttatggttatggtggttatggttgttatggttatggttatggttatggttatac

SEQ ID NO: 58 - DNA, 148 bp, Bos taurus
gtagttgtcctgatggttatagttatggttatggttgtggttatggttatggttgtagtggttatgattgttatggttatggtggttatggtggttatggtggttatggttatagtagttatagttatagttatacttacgaatatac

SEQ ID NO: 59 - DNA, 14 bp, Bos taurus
gaactcggtggggc

SEQ ID NO: 60 - DNA, 54 bp, Bos taurus
actatgcagacttccatctctggagccaggctgccctgggcaccgtctcctcag

SEQ ID NO: 61 - DNA, 56 bp, Bos taurus
ctgctgggacttggatctctggggccagcgcaccccggtcaccatgtccttgggga

SEQ ID NO: 62 - DNA, 50 bp, Bos taurus
caatgcttttgactcctggggccagcgcacccccatctccatctcctcag

SEQ ID NO: 63 - DNA, 47 bp, Bos taurus
actattcgacaactggggcccaggaatccaaaacaccgtctcctcag

SEQ ID NO: 64 - DNA, 50 bp, Bos taurus
taacaactggctcaagcactggggtcaggaagcctgggcactgtctgctc

SEQ ID NO: 65 - DNA, 54 bp, Bos taurus
tttactatggtatagacgcctggggccgagggctcagggtcaccgtctcctcag

SEQ ID NO: 66 - DNA, 63 bp, Bos taurus
actatgctgacttccatctctgtggccaggctgccctgggcaccgtctcctcagctgaatctg

SEQ ID NO: 67 - DNA, 56 bp, Bos taurus
ctgctgggacatggatctctggggccagcgcaccccggtcaccgtgtccttgggga

SEQ ID NO: 68 - DNA, 50 bp, Bos taurus
caatgcttttgactcctggggccagcgcgccccggtctccatctcctcag

SEQ ID NO: 69 - DNA, 48 bp, Bos taurus
actacgtcgatgcctggggccaaggactcctggtcaccgtctcctcag

SEQ ID NO: 70 - DNA, 50 bp, Bos taurus
taacaactggctcaagcactggggtcgggaagcctgggcactgtctgctc

SEQ ID NO: 71 - DNA, 54 bp, Bos taurus
attactatagtatatatgtttgcggccgagggatcgaggtcaccgtctcctcag

SEQ ID NO: 72 - DNA, 287 bp, Bos taurus
gacatccaggtaacccagtctccatcctccttgtctgcatctctaggagacagagtctccatcacttgccaggccagtcagagcattgacactaaattagcctggtatcaacagaaaccagggaaagctcctaagctcctcatctatgcaatacccaggtcgccttcctggttcccttcccagttcagtggcagtggatttggggcagatttcaccctcaccatcagcagtctgaaggctgatgatattgcaacttactactgtcagcaggatcacggtttacctac

SEQ ID NO: 73 - DNA, 287 bp, Bos taurus
gacatccaggtgacccagtctccctcctacctgtctgcttctctaggagacagagtctccatcacttgccaggccaatcagagcgttagccactacttaaactggtatcaacagaaaccaggggaagctcctaagctcctgatctattatgcaaccagccggtacaccagagtcccatcccgattcagtggcagtggatctgggacagatttcaccctcaccatcagcagcctggaggctgacgatgctgcaaattattactgtcaacaggattatagtacacctcc

SEQ ID NO: 74 - DNA, 286 bp, Bos taurus
ggcatccagatgactcagtctccatcctccttgtctgcctctctaggagacagagcatccatcatttgctgggccaattaaagcattagcaaatggttagacagatatgagcagaaaccagggcaagttcctaagctcctgttctatgcagcatccaatttgggaactggggtcccatcccggttcagtggcagtagatctgggacagatttcactgtcaccactctcacctggaggctgaagatgctgcaacttattactgtctacaaactgatagtacacctcc

SEQ ID NO: 75 - DNA, 285 bp, Bos taurus
gacctccagatgattcagtctctatcttccctgtctgcatctctaggagacagagtctccatcacttgtcgggccagtcaaagcgttagaaataatttacagtggtatcaagagaaaccagggaaagctcctaagttcctcatctatgacagaaccagtgtgtacacaggggtcccatcccatttcagtggcagtggatctgggacagattataccttcaccaccagcagcctgggctgatgattttgcaacttattactgtaaacaggataacagtagacctcc

SEQ ID NO: 76 - DNA, 283 bp, Bos taurus
gacctccagatgacccagtctccatcctccctgtctgcatctctaggagacagaatctccatcacttgccgggccagagcgttagcaactacttagcctggtatcaacagaaaccagggaaagctcctaagctcctgatctatcacgaatccagattgcacacaggggtcccatcccggttcagtggcagtggatgtgggacagattacaccctcaccatcagcaggctggagtctgacgatgctgcaaattattactgtcagcagtataatagtacacctcc

SEQ ID NO: 77 - DNA, 302 bp, Bos taurus
gatgttgtgctgacccagactccactctccctgtctatcatccctggagagatggcctccatctcctgcaagtctagtcagagcctggtacacagtgatggaaaaacctatttgaattggattcaatataaaccaggccaatcaccacagggtctgatctatcaggtttccaaccgttactctggggtctcagacaggttcactggcagtgggtcagggacagatttcacacttacaatcagcagagtgcaggctgaggatgctggagtctattactgttaccaaggtacagaagatcctcc

SEQ ID NO: 78 - DNA, 302 bp, Bos taurus
gctactatgcagacccagactctacgctccctgtctgtcatcccgggagagatggcctccatctcctgcagagccagtcagagcgttcaaaatagatatggagacaattttttgcactggtatgtgcagaagcccagccagtctccacagctcctgatttatagggcttctaactgggagtcttgggtcccagacaggttcacaagcagtgggttgggaacacatttcatcctcataatcagcagggtggagtctgaggatgctggagtttattactgccagcagagtttacaagcacctcc

SEQ ID NO: 79 - DNA, 302 bp, Bos taurus
gatgttgtgctgacccagactcccctctccctgtctgtcatccctggagagacggtcaccatctcctgcaagtctactcagagtctgaaatatagtgatggaaaaacgtatttgcaatggtttcaacataaaccaggccagtctccacggctattgatctatcagatttccaaccgttacactggggtcccagacaggttcactggcagtgggtcagagacagatttcacacttacaatcagcagtgtgcaggctgaggatgctggagtctattactgtcttcaaagatcatatgctcctcg

SEQ ID NO: 80 - DNA, 303 bp, Bos taurus
ggctattatgcagaaccaactatacgctccctgtctgtcatccctggagagactgccttcatctcctgcagagccagtcagagcattcaatatagatagggagacaatttttttgcactggtatgtgcagaagcccagccagtctccacagctcctgatttatagggcttctaactgggagtcttgggtcccagacaggttcacaagcagtgggttgcgaacagatttcatcctcataatcagcagggtggaggctgaggatgctggagtttattactgccagcagagtttacaagcacctcc

SEQ ID NO: 81 - DNA, 302 bp, Bos taurus
gatgttgtgctgacccagactcccctctccctgtctgtcatccctggagagacggtctccatctcctgcaagtctactcagagtctgaaatacagtgatggaaaaacctatttgtaccggcttcaacataaaccaggccaatcaccacagagtttgatctattatgtttccaaccgttacactggggtcccagacaggttcactggcagtgggtcagagacagatttcacacttacgatcagcagtgtgcaggctgaggatgctggagtctattactgttttcaaggcacacaggttcctcc

SEQ ID NO: 82 - DNA, 303 bp, Bos taurus
gctataaggcagacccagactctacgctccctgtctgtcatccctggagagacggcctccgtctcctgcagagccagtcagagcgttcaaaatagatatggagacaatttttttgcattggtatgtgcagaagcccagccagtctccacagctcctgatctatggagcttctaaccaggcctctggagtctgagacaggttcactggcagtgggtcagggacagacttcaccctcaaaagcagcagggtcggggctgaggatgctggagtttattattgccaccaaagtaaagaaactcctcc

SEQ ID NO: 83 - DNA, 302 bp, Bos taurus
gatgttgtgctgacccagactcccctctccctgtctgtcatccctggagagacggtctccatctcctgcaagtctactcagagtctgaaatatagtgatggaaaaacctatttgcgttgggttcaacataaaccaggccaatcaccacagggtgtgatctatcaggtttccaaccgtaatactggggtcccagacaggttcactggcagtgggtcagaaacagatttcacacttacaatcagcagtgtgcaggctgaggatgctggagtctattactgttttcaaggtacatatgaacctcc

SEQ ID NO: 84 - DNA, 303 bp, Bos taurus
gctataatgcagacccagactctacgctccctgtctgtcatccctggagagacggcctccatctcctgcagagccagtcagagcgttcaaaatagatatggagacaatttttttgcattggtatgtgcagaagcccagccagtctccacagctcctgatctatggagcttttaaccaggcctctggagtctgagacaggttcaccggcagtgggtcagggacagatttcaccttcaaaaccagcagggtgggggctgaggatgctggagtttattattgccaccaaagtaaagaaactcctcc

SEQ ID NO: 85 - DNA, 299 bp, Bos taurus
gatgttgtgctgacccagactcccctctccctgtctgtcatccctggagagacggtctccatctcctgcaagtctactcagagtctgaaatatagtggaaaaacctatttgcgttggcttcaacataaaccaggccaatcaccacagagtctgatctatcaggtttccaaccgttacactggggtcccagacaggttcactggcagtgggtcagagacagatttcacacttacgatcagcagtgtgcaggctgaggatgctggagtctattactgtgttcaagagacacatgatcctcg

SEQ ID NO: 86 - DNA, 301 bp, Bos taurus
gctattgttctgacccagactccacgctccctgtctgtcatccctggagagacggcctccatctcctgcagatccagtcagagcattcaaaatagatatggagacaatcttttgcactggtatgtgcagaagcccagccagtctccacagctcctgatctatggaacttctaaccaggcctctggagtctgagacaggttcaccggcagtgggtcagggacagatttcaccctcaaaaccagcagggtggaggctgaggttgctggagtttattattgcaggaaagtaaagaaactccttc

SEQ ID NO: 87 - DNA, 302 bp, Bos taurus
gatgtagtgctgacccagactccactctccttgtctgtcatccctggtgagacggcctccatctcctgcaagtcaagtcagagcctcctgcatagtgatggaaaaacctatttgaactggtttcaacataaaccaggccagtctccacagtgactgatctatcaggcttccaaccgtgacactggggtctcagagaggttcactggcagtgggtcagggacagatttcacacttaaaatcagcagagtgcagattgagtatgctggcatctattactgttttcagcatacatatgatcctcc

SEQ ID NO: 88 - DNA, 302 bp, Bos taurus
gacattgtgctgacccagactccactctccttgtctgtcttccctggagagacggcgtccatctcctgcagaaccagtcagagccttgaagatagttatggagacacttatttgagttggcacttgcagaagcctagccagtctccacagcttctgatctatttggtttccaatagagcctctggggtcccagacaggttcactggcagtgggtcaggaacagatttcacctttaaaatcagcagggtggaggctgaggatgctggagtttattactgccaacagagtatacaagcacctcc

SEQ ID NO: 89 - DNA, 286 bp, Bos taurus
gaaattatgttaacgcagtctccagcctccctgtctttgactccaggggaaatagccaccctcacctgcagggccagtcaaagtattagtagctacttaagactggtaccagcagaagcctgggaaggcccccagattcttcatctatgctgcctccagcagggcctctggcatcccagcccggttcggtgacagttgggtcagggacagactttactctcaccatcagcagcctggagcctgaagatgctgcagttcattcctagtgctagcataatagcgggaa

SEQ ID NO: 90 - DNA, 287 bp, Bos taurus
gaggctgtgctctaccagactccagcctacatcgctgcatccctaggagagagcatctccatcacttgcagagccaatcaaagcattagtgattacttaagctggtataagcagaaacctggccaggctcctatgattctcatctatgatgctgataatcgttataatggtgtcccagagaggttcactgcgactcaatctgagacagaatttgttttcacaatcagccaagtagaggctgatgatgctgccatgtattactgccagcaggattatgcacttcctcc

SEQ ID NO: 91 - DNA, 138 bp, Bos taurus
gacatcatgatgacccagtctcgaagttccttggctgagtctgcaggagaggaaggtcatcatcatctacagatccagccagaatcttctatacttcaaccagaaaacctagtttgcctggtaccagcagaaactgtg

SEQ ID NO: 92 - DNA, 285 bp, Bos taurus
gctgctgtactgactccatctcctccctctggcctgtggccatggagggagcgtcgccatctcctgaaggccatctcttcccatccacagtaatggacacacctgcccgccgtgattcgggcacaaaccacacactctcctcaaccactgatcatagggattcccaggctcctgaggtcccagcctggctcagtgattgtgggtctggatggatttcacacttacactcaccagggtggcgtcccttcatgtgacttctgtgtacagaaccctcactgggaccac

SEQ ID NO: 93 - DNA, 285 bp, Bos taurus
actgctgtgctgactccatctctccctctggcctgtggccatggagggagcgtcgccatctcctgaaggccatctcttctcatccacagtaatggacacaccttcccgccatgcttctggcacaaaccacacactctcctcaaccactgaccatagagggtcaccaggctcttgaggtcccagcctggctcagtgattgtgggtctggatagatttcacactcacactcaccagggtggggtccctacatgtgacttctgtgcacagaaccctcacttggaccac

SEQ ID NO: 94 - DNA, 286 bp, Bos taurus
gctgctgtgctgacttcatctctccctctggcctgtggccatggagggagcatcgccatctcctgaaggccatctcttctcatccacagtaatggacacacctgcccgccatgcttctggcaaaaaccacacactctcctcaaccactgatcataggtggtccccaggcttcaggggtccaagcctggctcagtgactgtgggtctgggacggatttcacacttacacttaccagggtggggtccctacatgtgacttctgtgcacagaaccctcactgggaccac

SEQ ID NO: 95 - DNA, 284 bp, Bos taurus
gctgaggagactccatctcctccctctggcctgtggccatggagggagcgccgccatctcctgaaggccatctcttctcatccacagtaatggacacacctgcccaccatgtttccggcacaaaccacacactctcctcaaccactgatcatagggcttccccaggcttcaggggtcccagcctggctcagtgactgtgggtctgggatggatttcacacttacactcaccagggtggggtctctacatgtgacttctgtgcacagaaccctcactgggaccac

SEQ ID NO: 96 - DNA, 294 bp, Bos taurus
gctgctgtgctgactccgtcccctccctctggtctgcagtcgtggaaagaggcatctccatctcctgcaaggccatcccatctcatccatagaaatgaatacacctgtcctccctccttccagaacaaaccacacactctcctcacccattgacataggggtcccccaggctcctggggtcccatcctggctcagtggccatggatctgggacggatttcacactcacactcaccactgtggagactggggaccctgaatgtgacttctgtgcacagagccttcaatgggaact

SEQ ID NO: 97 - DNA, 38 bp, Bos taurus
atggacgttaggtcaaggaaccaagctggaagtcaaac

SEQ ID NO: 98 - DNA, 39 bp, Bos taurus
taaatactttcggccaaggaaccaaggtagagatcaaaa

SEQ ID NO: 99 - DNA, 38 bp, Bos taurus
gttcactttcgggccaaggaccagagtggagatcaaat

SEQ ID NO: 100 - DNA, 38 bp, Bos taurus
aattacgttcggcggcgggaccaaggtggaaatcaatc

SEQ ID NO: 101 - DNA, 38 bp, Bos taurus
gatcatctttggccaagggacacgtctggagattagac

SEQ ID NO: 102 - DNA, 296 bp, Bos taurus
caggctgtgctgactcagccgccctccgtgtccgggtccctgggccagacggtcaccatctcctgcaccggaagcagcaacaacatcgggattttgggtgtgagctggtaccaacagatcccaggatcggcccccagaaccctgatctataatagtaacaaacgaccctcgggggtccccgaccgattctctggcaccaagtccggcaacacaggcaccctgaccatcgcttcgctccaggctgaggacgaggctgattattactgtgcgtctgctgacctcagtcttactagtcc

SEQ ID NO: 103 - DNA, 291 bp, Bos taurus
caggctgtgctgactcagcagccctccgtttccgggtccctgggccagagggtctccatctcctgctctggaagcagcagcaacattgggcatggttatggtacctggtaccaacagatcccaggatcggcccccagaatgctcatctatggtgcgaccagtcgagcctccggtccccgaccgattctccggctccaggtctggcaacacagcgactctgaccatcagctcgctccaggctgaggatgaggcggattatttctgtgcagcttatgacagtagcagtggtcc

SEQ ID NO: 104 - DNA, 299 bp, Bos taurus
caggatgtgctgactcagccgtcctccgtgtccgggtccctgggtcagaaggtctccatcacctgctctggaagcagcagcaacgttggatatgccaattatgtgagctggcaccaacagaaaccaggatcggcccccagaaccctcatctatggtgcgaccagtcgagcctcgggggtccctgaccaattctccggctccaagtctggcaacacagcgactctgaccatcagctcgctccagcctgaggacgaggctgattattactgttcatcttatgacagtagcagcaatattgg

SEQ ID NO: 105 - DNA, 291 bp, Bos taurus
caggctgtgctgactcagccgccctccgtgtctgggactttgggtcagagggtcaccctctcctgcactggaagcagcagcaacactggggtctttatgtgagctggtaccaacagctcccaggaaggcccccagagtcctgacctatgaaaatagcaaacgaacctcaggactcccagattgattctctggctccaagtctggcagctcggccgcactgaccacctcagttcagtctgaggacgacactgattattactgtttctcatgggctgatggattgaaagtttg

SEQ ID NO: 106 - DNA, 292 bp, Bos taurus
caggctgtgctgactcagccgccctccgtgtccaggactttgggtcagagggtcaccctctcctgcactggaagcagcaacaaccctggggttattctgtgagctggtaccaacagctcccaggaaaggcccccacacttctcatctatgaaaatagcacacgaccctcagcactcccagattgattctctggctccaagtctggcaagtcggtctctctgaccacctcagttcagtctgaggacgacactgattattactgtttctcatgggctgacggattgaaagtttg

SEQ ID NO: 107 - DNA, 296 bp, Bos taurus
caggctgtgctgactcagccgtcctccgtgtccggctccctgggccagagggtctccatcacctgctctggaagcagcaacaacatcggtagttatggtgtgggctggtaccaacaggtcccaggatcgggcctcagaaccatcatctatggtagtagcagtcgaccctcgggggtccccgaccgattctccggctccaagtctggcaacacagccaccctgaccatcagctcgctccaggctgaggacgaggcggattatttctgtgcaactgttgactacagtagcagtactgt

SEQ ID NO: 108 - DNA, 287 bp, Bos taurus
caggctatgctgactcagctgccctccatgtccgggactttgggtcagagggtcaccctctcctgcactgaaagcagcagcaaccctggggtctttatgtgagctggtaccaacagctcccaggaaaggcccccagagtcctgacctgtgaaaatagcaaacgaccctcaggggtcccagattgattctctggctccaagtctggcaacagcctctcttaccacctcagttcatgctgaggatactgattactactgtttctcatgggctgacggcttgaaagtttg

SEQ ID NO: 109 - DNA, 295 bp, Bos taurus
caggctgtgctgactcagccgtcctccgtgtccgggtccctgggccagagggtctccatcacgtgctctggaagcagcagcaacgttggatatggcaattatgtgagctggttccaagacatcccaggatcggcccccagaaccctcatctatggtgacaccagtcgagcctcgggggtccccgaccgattctccggctccaggtctgggaacacagccaccctgaccatcagctcgctccaggctgaggacgaggcagattatttctgtgcatcttatcagagtggtaacacag

SEQ ID NO: 110 - DNA, 295 bp, Bos taurus
caggctgtgctgactcagccatcatccgtgtccgggtccctgggccagagggtctccatcacctgctctggaagcagcagcaatgttggaaatggatatgtgagctggtaccaactgatcccaggatcggcccccagaaccctcatctatggtgacaccagtcgagcctcgggggtccccgaccgattctccggctccaggtctggaacacagccaccctgaccatcagctcgctccaggctgaggacgaggcagattatttctgtgcatctgctgaggatagtagcagtaatgc

SEQ ID NO: 111 - DNA, 291 bp, Bos taurus
caggctatgctgactcagccgccctccatgttcgggactttgggtcagagggttaccctctccttcactggaaggagcagcaacactgggggtctttatgtgagctggtaccaacagctcccaggaaaggcccctagactcctgacatatgaaaatagcaaacgaccctcaggggtcccagattgattctctggctccaagcctgccaactcagcctctctgaccacctcagttcatgctgaacgatactgattattactgtttctcatgggctgatggcttgaaagtttg

SEQ ID NO: 112 - DNA, 295 bp, Bos taurus
caggctgtgctgactcagccgtcctccgtgtccgggtccctgggccagagggtctccatcacctgctctggaagcagcagcaacgttggaactggcaattatgtgagctggttccaacagatcccaggatcggcccccagaaccctcatctatggtgcgaccagtcgagcctcgggggtccccgaccgattctccggctccaggtctgggaacacagccaccctgaccatcagctcgctccaggctgaggacgaggcagattatttctgtgcatcttatcagagtggtaacacag

SEQ ID NO: 113 - DNA, 299 bp, Bos taurus
caggctgtgctgactcagccgtcctccatgtccgggtccctgggccagagggtctccatcaccagctctggaagcagcagcaacgttggatatggcatttatgtgaaccagtaccaaaaaatcccaggatcggcccccagaaccctcatctatggtgccaccagtcgagcctcgggggtccccgaccgattctccggctccaggtctgggaacacagccaccctgaccatcagctcgctccaggctgagaacgaggcagattatttctgtgcagcttatgacagcagtagcagtgatgg

SEQ ID NO: 114 - DNA, 299 bp, Bos taurus
caggctgtgctgactcagccgtcctccgtgtccgggtccctgggccagagggtctccatcacctgctctggaagcagcagcaacgttgggcttggtaattatgtgagctggttccaacagatcccaggatcggcccccagaaccctcatctatggtgcgaccagtcgagcctcgggggtccccgaccgattctccggctccaggtctgggaacacagccaccctgaccatcagctcgctccaggccgaggacgaggcggattatttctgtgcatctcctgacagtagtagcagtagtta

SEQ ID NO: 115 - DNA, 291 bp, Bos taurus
caggctatgctgactcagccgccctccatgttcgggactttgggtcagagggttaccctctccttcactggaaggagcagcaacactgggggtctttatgtcagctggtaccaacagctcccaggaaaggcccctagactcctgacatatgaaaatagcaaacgaccctcaggggtcccagattgattctctggctccaagcctggcaactcagcctctctgaccacctcagttcatgctgaacgatactgattattactgtttctcatgggctgatggcttgaaagtttg

SEQ ID NO: 116 - DNA, 295 bp, Bos taurus
caggctgtgctgactcagccgtcctccgtgtccgggtccctgggccagagggtctccatcacgtgctctggaagcagcagcaacgttggatatggcaattatgtgagctggttccaagagatcccaggatcggcccccagaaccctcatctatggtgacaccagtcgagcctcgggggtccccgaccgattctccggctccaggtctgggaacacagccaccctgaccatcagctcgctccaggctgaggacgaggcagattatttctgtgcatcttatcagagtggtaacacag

SEQ ID NO: 117 - DNA, 299 bp, Bos taurus
caagctgtgctgactcaaccgccctccatgtctgggtccctgggccagagggtctccatcacctgctctggaagcagcagcaacgttggaactggcaattatgttggctggtaccaaatgatcccaggatcggcccccagaaccctcatctaccgtgctaccagtcgactctcgggggtccccgactgattctccgtctccaggtctgggaacacagccaccctgaccatcagctcgcaccaggctgaggacgaggctgattattactgtgtatcttaggacagcagtatcagtggtgc

SEQ ID NO: 118 - DNA, 296 bp, Bos taurus
caggctgtgctgactcagccatcatccgtgtccgggtccctgggccagagggtctccatcacctgctctggaagcagcagcaatgttggaaatggatatgtgagctggtaccaactgatcccaggatcggcccccagaaccctcatctatggtgacaccagtcgagcctcgggggtccccgaccgattctccggctccaggtctgggaacacagccaccctgaccatcagctcgctccaggctgaggacgaggcagattatttctgtgcatctgctgaggatagtagcagtaatgc

SEQ ID NO: 119 - DNA, 291 bp, Bos taurus; identical to SEQ ID NO: 111

SEQ ID NO: 120 - DNA, 299 bp, Bos taurus
caagctgtgctgactcaaccgccctccatgtctgggtccctgggccagagggtctccatcacctgctctggaagcagcagcaacgttggaactggcaattatgttggctggtaccaaatgatcccaggatcggcccccagaaccctcattgaccgtgctaccagtcgactctcaggggtccccgactgattctccgtctccaggtctgggaacacagccaccctgaccatcagctcgcaccaggctgaggacgaggctgattattactgtgtatcttacgacagcagtatcagtggtgc

SEQ ID NO: 121 - DNA, 296 bp, Bos taurus; identical to SEQ ID NO: 118

SEQ ID NO: 122 - DNA, 291 bp, Bos taurus; identical to SEQ ID NO: 111

SEQ ID NO: 123 - DNA, 295 bp, Bos taurus
caggctgtgctgactcagccgtcctccgtgtccgggtccctgggccagagggtctccatcacctgctctggaagcagcagcaacgttggaactggcaattatgttggctggttccaacagatcccaggatcagcccccagaaccctcatctatggtgcgaccagtcgagcctcgggggtccccgaccgattctccggctccaggtctgggaacacagccaccctgaccatcagctcgctccaggctgaggacgaggcagattatttctgtgcatcttatcagagtggtaacacag

SEQ ID NO: 124 - DNA, 291 bp, Bos taurus
caggctgtgctgactcagccgccctccgtgtctgggactttgggtcagagggtcaccctctcctgcactggaagcagcagcaaccctggggtctttatgtgagctggtaccaacagctcccaggaaggcccccagagtcctgacctatgaaaatagcaaacgaccctcaggactcccagattgattctctggctccaagtctggcagctcggccgcgctgaccacctcagttcagtctgaggacgacactgattattactgtttctcatgggctgatggcttgaaagtttg

SEQ ID NO: 125 - DNA, 296 bp, Bos taurus
caggctgtgctgactcagccatcatccgtgtccgggtccctgggccagagggtctccatcacctgcaccggaagcagcagcaatgttggaaatggatatgtgagctggttccaacagatcccaggatcggcccccagaaccctcatctatggtgacaccagtcgagcctcgggggtccccgaccgattctccggctccaggtctgggaacacagccaccctgaccatcagctcgctccaggctgaggacgaggcagattatttctgtgcagctggtgacagcagtagcagtaatgc

SEQ ID NO: 126 - DNA, 291 bp, Bos taurus
caggctatgctgactcagccgccctccgtgtttgggactttgggtcagagggttaccctctccttcactggaaggagcagcaacactgggggtctttatgtgagctggtaccaacagctcccaggaaaggcccctagactcctgacatatgaaaatagcaaacgaccctcaggggtcccagattgattctctggctccaagcctggcaactcagcctctctgaccacctcagttcatgctgaatgatactgattattactgtttctcatgggctgatggcttgaaagtttg

SEQ ID NO: 127 - DNA, 298 bp, Bos taurus
caggctgtgctgactcagccatcatccgtgtccgggtccctgggccagagggtctccatcacctgctctggaagcagcagcaatgttggaaatggatatgtgagctggtaccaactgatcccaggatcggcccccagaacccttcatctatggtgacaccagtcgagcctcgggggtccccgaccgattctccggctccaggtctgggaacacagccacccctgaccatcagctcgctccaggctgaggacgaggcagattatttctgtgcatctgctgaggatagtagcagtaatgc

SEQ ID NO: 128 - DNA, 298 bp, Bos taurus
caagctgtgctgactcaaccgccctccatgtctgggtccctgggccagagggtctccatcacctgctctggaagcagcagcaacgttggaactggcaattatgttggctggtaccaaatgatcccaggatcggcccccagaaccctcatctaccgtgctaccagtcgactctcggggtccccgactgattctccgtctccaggtctgggaacacagccaccctgaccatcagctcgcaccaggctgaggacgaggctgattattactgtgtatcttaggacagcagtatcagtggtgc

SEQ ID NO: 129 - DNA, 293 bp, Bos taurus
caggctgggctaactcagccggcctccgtgttcaggactttgggtcagagggtcaccatctcttgtactggaagcagcaacaacattgggggttattatgtgagctggtaccaacagctcccaggaaaggcccccagactcctgacctatgaaattagcaaacgacccccaggggtcccagatcgagtctctggctccaagtctggcaactcagcctctctgaccagctcagttcatgctgaggacgacactgattattactgtttctcatgggctgacggcttgaaagtttg

SEQ ID NO: 130 - DNA, 299 bp, Bos taurus
caggctgtgctgacccagccgccctccgtgtccgggtccctgggccagagggtgaccatctcctgcactggaagcagcagcaacatcggtggtggtaattgtgtgggctggtaccaacagatcccaggatcggcccccaaaaccctcatctataggagtaccagtcgaccctcgggggtcccagaccgattctccggctccaggtctggcaacacggccaccttgaccatcagctcgctccaggccgaagacgaggcggattactactgtgcaacttacgaaagtagtagttatcatgg

SEQ ID NO: 131 - DNA, 291 bp, Bos taurus
caggctatgctgactcagccgccctccgtgttcgggactttgggtcagagggttaccctctccttcactggaaggagcagcaacactgggggtctttatgtcagctggtaccaacagctcccaggaaaggcccctagactcctgacatatgaaaatagcaaacaaccctcaggactcccagattgactctctggctccaagcctggcaactcagcctctctgaccacctcagttcatgctgaacgatactgattattactgtttctcatgggctgacggcttgaaagtttg

SEQ ID NO: 132 - DNA, 236 bp, Bos taurus
acctgctctggaagcagcaacaacatcggtagatatggtgtgggctggtaccaacaggtcccaggatcgggcctcagaaccatcatctatggtagtagcagtcgaccctcgggggtccccgaccgattctccggctccaagtctggcaacacagccaccctgaccatcagctcgctccaggctgaggacgaggcggattatttctgtgcaactggtgactacagtagcagtactgt

SEQ ID NO: 133 - DNA, 299 bp, Bos taurus
caggctgtgctgacccagccgccctccgtgtccgggtccctgggacagagggtgaccatctcctgcactggaagcagcagcaacatcggtggtggtaattatgtgggctggtaccaacagatcccaggatcggcccccaaaaccctcatctataggagtaccagtcgaccctcgggggtcccagaccgattctccggctccaggtctggcaacacggccaccttgaccatcagctcgctccaggccgaagacgaggcggattactactgtgcaacttacgaaagtagtagttatcatgg

SEQ ID NO: 134 - DNA, 293 bp, Bos taurus
caggctgtgctgactcagctgccctccgtgttcaggactttgggtcagagggtcaccatctcttgtactggaagcagcaacaacattgggggttattatgtgagctggtaccaacagctcccaggaaaggcccccagactcctgacctatgaaattagcaaacgacccccaggggtcccagatcgagtctctggctccaagtctggcaactcagcctctctgaccagctcagttcatgctgaggacgacactgattattactgtttctcatgggctgacggcttgaaagtttg

SEQ ID NO: 135 - DNA, 299 bp, Bos taurus
caggctgtgctgactcagccgccctccgtgtccgggtccctgggccagagggtgaccatcacctgcaccggaagcagcagctacgtttcgcgtggcaatcatgtgagctggtaccaactgatcccaggattggcccccaaaaccctgatctataatagtaacaaacgaccctcgggggtccctgaccgattctctggcaccaagtccggcaacacaggcaccctgaccatcgcttcgctccaggctgaggacgaggctgattattactgtgcgtctgctgacctcagtcttactggtcc

SEQ ID NO: 136 - DNA, 297 bp, Bos taurus
cagtctggcctgactcagccttcctcagtgtctgggaatctgggacagacggtcaccatctcctgtgctgggaccagcagtgatgtaggggcttataatggtgtgggctggtaccaacagctcccgggctcagcccccaaaactctgatctataatctcaacaaacggtcctcagggatccctgctcggttctctggctccaagtctgggaacacagccaccctgaccatctctgggctccaggctgaggacgaggccgactattactgtagctcatataaaagtggtggtagtgtg

SEQ ID NO: 137 - DNA, 297 bp, Bos taurus
cagtctagcctgactcagccttcctcagtgtctgggaatctgggacagacggtcaccatctcctgtgctgggaccagctgtgacgtagggagttataatggtgcgggctggtaccaacagctcccgggctcagcccccaaaactctgatatgtaatgtcagcaaacggccctcagggatccctgactggttctctggctccaagtccggaaacacagccaccctgaccatctctgggctccaggctgaggacgaggctgattactattggagctctcctagaagtgatagcactgtg

SEQ ID NO: 138 - DNA, 295 bp, Bos taurus
cagtctggcctgactcagcctccctcagtgtctgggaatctgggacagacggtcaccagctcctgttctgagaccagcagtgacatcatggttataactctgtagattggtactggcagcacttgggcacggccccacactactgatttatgctgtcagtaaacgaccctcagggatccctgatcgcttctctggctccaagcctggacacacagcctccctgactgtctctgggctccaggctgaggacgaggctgattatcactgtggctcagacagaagcagcaaccacttg

SEQ ID NO: 139 - DNA, 297 bp, Bos taurus
cagtctggcctgactcagccttcctcagtgtctgggaatctgggacagactgtcatcacctcctgtgctgggaccagcagttatgtagggagttataatggtgtgggctggtaccaacagctcccgggctcagcccccaaaactctaatatataatgtcagcaaacggccctcaggaatccctgaccgcttctctggctccaagtccgggaacacagccaccctgaccgtctctgggctccaggctgaggacgaggccgactactactgtagctcatataaaagtggtggtagtgtg

SEQ ID NO: 140 - DNA, 291 bp, Bos taurus
tcctacgagctgactcagtcacccccggcatcgatgtccccaggacagacggccaggatcacgtgtggggggcccagcgttggaggtgaaaatgttgagtggcaccagcagaagccaggccaggcccgtgcgctggtcacctatggtgacgataaccgacccacgggggtccctgaccagttctctggcgccaactcagggaacatggccaccctgaccatcagcggggcccgggccaaggatgaggccgactattactgtcagctgtgggacagcagcagtaacaatcct

SEQ ID NO: 141 - DNA, 285 bp, Bos taurus
tcttctcagctgactcagccgcctgcggtgtccgtgtccttgggacagacagccagcatcacctgccagggagacgacttagaattgcttagtgcccactggtaccagcagaagccgggccaggcccctgtgctggtcatttatgcagatgacaacctggcctcagggatccctgaccggttctctggctccaaatcagacaccacggccaccctgaccattcgcggggcccaggccgaagacgaggccgactattattgtcagtcagctgatatcagtggtgtt

SEQ ID NO: 142 - DNA, 291 bp, Bos taurus
tcctatgaactgacacagttgacttcagtgtcagtggccttgggacagacggccaagatcacctgctcgggggagctgctggatgaacaatatactcagtggtaccagcagaagccgggccaggcccctaagctggtcatttataaagacagtaagcggcgctcagggatccctgaccagttctctggctccagctccggcaaaacagccatcttgaccatcagtggggtccgtgccgaggatgaagccgactattactgtctgtcgtgggacagtggcagttacaatgtt

SEQ ID NO: 143 - DNA, 288 bp, Bos taurus
tcctatgaactgacccagccgacttcagtgtcagtggccttgggacagacggccaagatcacctgctcgggggacctgctggatgaacaatatactcagtggtaccagcagaagccgggccagggccctgtgagggtcatttataaagatagtgagcggccctcagggatctctgaccggttctctggctccagctcaggcaaaacagccacgctgaccatcagcggggcccagaccgaggacgaggccgactattactgtcagtcagctgacagcagtgataatcct

SEQ ID NO: 144 - DNA, 288 bp, Bos taurus
tcttctcagctgactcagccgcctgcggtgtccgtgtccttgggacagacggccagcatcacctgccagggagacgacttagaaagctattatgctcactggtaccagcagaagccaagccaggcccctgtgctggtcatttatgagtctagtgagagaccctcagggatccctgaccggttctctggctccagctcagggaacacggccaccctgaccatcagcggggcccagactgaggacgaggccgactattactgtcagtcatatgacagcagcggtgatcct

SEQ ID NO: 145 - DNA, 308 bp, Bos taurus
cagcctgtgctgactcagccagccaccctctctgcgtctctgggagcatcagccaaactcaccggcaccctgagcagtggctacaatgttggcagctactacataaactggtaccagcagaagccagggagtcctccctggtacccctgtattgttactcagactccaataagcaccagggttccagggtccccagccacttctttggatccaaagacacctcggtgaaggcagggctcctgctaatctcggctacaggctgaggacaaggctgactattactctgctacatattgcagtagtactaa

SEQ ID NO: 146 - DNA, 315 bp, Bos taurus
cagcgtgtgctgactcagccggcctccccctctgcgtctccgggagcatcagccagactcccagactgcaccctgaacagtgggtctatcttggtggctagcaaatgtcctgtttccagcagaagccagggagccctccccaggacctcctgatgttcaagtcagactccgataagccccagggctccggggtccccagtcacttctctggatccaaggctgcctcagccaatgcagggcccccgttcatctctgggctgcagcctgaggctgaggctgattataactgctactgtccccaaaacactgcattca

SEQ ID NO: 147 - DNA, 285 bp, Bos taurus
cagcctgtgctgactcagtcagactccctgtctgcatctctgggagcatcagccagactctcctgcaccctgagcaatggctataacattggcagcttgtctataacctggtgccagcagaagccagggagtcctccccggtacctcctgtcctacaactcagattcccaaaagctccagggctccggggtccccagacacttctctggatccaaagacacctcgtccaacgcggggctcctgctcatctctgggctgcagacgggggacgaggctgtaggttcc

SEQ ID NO: 148 - DNA, 285 bp, Bos taurus
cagcctgtgctgactcagtcagactccctgtctgcatctctgggagcatcagccagactctcctgcaccctgagcaatggctataacattggcagcttgtctataacctggtgccagcagaagccagggagtcctccccggtacctcctgtcctacaactcagattcccaaaagctccagggctccggggtccccagacacttctctggacccaaagacacctcgtccaacgcggggctcctgctcatctctgggctgcagacggaggacgaggctgtaggttcc

SEQ ID NO: 149 - DNA, 317 bp, Bos taurus
cagcctgtgctgactcagccgtcgccgtctctgcgtctctgggagcatcagccagactctcctgcaccctgagcagtggctacaatgttagcaactatagcaatatactggtatcagcagaaggcagggaaccctctccggtacctcctgaggttcaaatcagactcggataaacaccagggctccggggtccccagccgcttctctggatccaaagatgcctcgaccaatgcagggctcctgctcatctctgggctgcagcccgaggacgaggccgactactactgtgctgtgtggcatggcgacactaacgctta

SEQ ID NO: 150 - DNA, 317 bp, Bos taurus
cagcctgtgctgactcagccagtcaccgtctctgcgtctctgggagcatcagccagactctcctgcaccctgagcagtggctacaatgttagcaactatagcatatactggtatcagcagaaggcagggaaccctctccggtacctcctgaggttcaaatcagactcggataaacaccagggctccggggtccccagccgcttctctggatccaaagatgcctcgaccaatgcagggctcctgctcatctctgggctgcagcccgaggacgaggccgactactactgtgctgtgtggcatggcgacactaacgctta

SEQ ID NO: 151 - DNA, 314 bp, Bos taurus
cagcctgtgctgactgagccggcatccccctctgcatatccaggagcatcagccagactcacctgcaccctgagcagtgggtaccgtgttggtggctaccaaatgtcctgtttccagcagaaggcagggagccctccctggtacctcctgatgttcaagtcagactcggataagccccagggctctggggtccccagtcacttctctggatccaaggctgcctcagccaacacagggctcctgctcatctccgggctgcagactcaggatgaggctgattataactgctactgtccccgaaacactggtattta

SEQ ID NO: 152 - DNA, 292 bp, Bos taurus
cagactgtggtccaggagccagcgctgtcagtgtgtccagtagggacggtcaccctcaccggtggactgagctctgggtcagtcactaccagtaactgcccagctggtaccagcagaccccgggccaggctccccgactgcttatctacagcacaagcagccgatattctggggtccctgctcacttctctggctccatctctggaaacaaatccaccctcaccatctcgggggcccagtccgaggtagaagccgactattactgtggtctgggaactggtagttacaatgc

SEQ ID NO: 153 - DNA, 292 bp, Bos taurus; identical to SEQ ID NO: 152

SEQ ID NO: 154 - DNA, 293 bp, Bos taurus
tagactgtggcccagaagccgtcacggccagtgtctccaggagagacggtcaccctcacctgtggactgagctctgggtcagtcacaaccagtaactaccctagctggttgcagcagaccccaggccaggctccctgactgcttttctatagcacaaacagtcgcccgtctggggtctctaattgcatctctggttccatctctgggaacaaagccaccctcaccatcacgggggcccagtccgaggacgaagccgattatcactgtggtctgggaactggtagttacaatgc

SEQ ID NO: 155 - DNA, 292 bp, Bos taurus
cagactgtggtccaggagccagcactgtcagtgtgtccaggagggacggtcaccctcacctgtggactgagctctgggtcagtcactaccagtaactgcccagctggtaccagcagaccccaggccaggctccccgactgcttatctacagcgcaagcagctgatattctggggtccctgcttacttctctggctccatctcgggaaacaaatccaccctcaccatctcgggggcccagtccgaggtagaagccgactattactgtggtctgggaactggtagttacaatgc

SEQ ID NO: 156 - DNA, 292 bp, Bos taurus
gcagcagtggcccagaagccgtcacggtcagtgtgtccaggaggcacggtcaccctcacctgtggactgagctctgggtcggtcactacaggtaaccacccagctggttccagcagaccccagtgcagcctcccggaactgtcaactacaacaccaacacccgtccctctggggtccctggtaacttctctggctcctcctctgggagcagatctgccctcaccatcacaggagaccagtccgaggacaaagccaactatcactgtgctctgggagctagtagttaaaatcc

SEQ ID NO: 157 - DNA, 299 bp, Bos taurus
cagattgtgatccaggaaccgtcactgtcagtgtctccaggagggacggtcaccctcacctgtggactgagctctgggtcagtcactacttacaacgaacccagctggtaccagcagaccccaggccaggctcccagaaatgttatctacaacacaaacacccgcacctctggggtccctgatcgcttctctgcctccatctctgggaacaaagccaccctcaccatcacgggggcccagcccaaggacgaggctgactatcactgcttgctgtaccagggcagtggtagttacagctg

SEQ ID NO: 158 - DNA, 293 bp, Bos taurus; identical to SEQ ID NO: 154

SEQ ID NO: 159 - DNA, 293 bp, Bos taurus
tagactgtggcccagaagccgtcacggccagtgtctccaggagagaaggtcaccctcacctgtggactgagctctgggtcagtcacaaccagtaactaccccagctggttgcagcagaccccaggccaggctccctgactgcttttctatagcacaaacagtcgcccgtctggggtctctaattgcatctctggttccatctctgggaacaaagccaccctcaccatcacgagggcccagcccaaggacgaagccgattatcactgtggtctgggaagtggtagttacaatgc

SEQ ID NO: 160 - DNA, 294 bp, Bos taurus
tagaactgtggcccagaagccgtcacggccagtgtctccaggagagaaggtcaccctcacctgtggactgacctctgggtcactcacaaccagtaactaccccagctggttccagcagaccccaggccaggctccctgattgctttcctatagcacaaacagtcgtccgtctggggtttctaattgcatctctggttccatctctgggaacaaaaccaccctcaccatcaaggtggcccagcccaaggacgaagccgattatcactgtggtctgggaactggtagttacaatgc

SEQ ID NO: 161 - DNA, 293 bp, Bos taurus
caatccgggctgactcaggaggcctccgtgtcacggtctctgggtcagtcggtcaccctcacctgcactgggagcagcaacaacgttggattctatggcgcgggctggtcccaacaccgcccaggtgctgcccccagaaccgtggtgctgggaagttctcgaccctcaggcctcccagcccggctctcgggctcctgttctggctccaccacctcactgagcatctctgggctccaggctgcggacgaggctgactattactgttccctgtgggcccgcagcctcagtgctcc

SEQ ID NO: 162 - DNA, 176 bp, Bos taurus
gtgtctttgtatcaggagaacccaggctctgccctaaaatctctgatttatgatgtcagtaaaaggtcctcaggggtcctgtttgcttctcaggctcaaactctgggaacaccctggccacctctgggctccaggctgactcttattgtggctcacatgaaagtggacgcaatttg

SEQ ID NO: 163 - DNA, 244 bp, Bos taurus
tatggacgctcagccacactcgcctgcctgggaacagcaacactgttggcaccaagggggcgacttggctgccgtctcagtcgtgctgagtcccaagctctgagcacaggagtcacaacccacccgcagggtctcagcgaggcctgagggctccgggtcaggtggggccacctgaccatctctgggctccagcctgacgccaaggctgattgttcctgctcagctgggactcagccctgctgtt

SEQ ID NO: 164 - DNA, 245 bp, Bos taurus
tgcaccctgagcagtgacatcagtgtcggctgctctgctgttactggaacaagcagcagccagggagccctcttcggtcctctggtcctaccactcagactccagtaagaaccaggctctggggtccccgtgggttttctggatccaaagatgccttggccaacgtggggctcctgctcgtctctgggctgcagcctgaggatgaggctgactctcaccatgcaggctggtgcaacagggcttct

SEQ ID NO: 165 - DNA, 245 bp, Bos taurus
tgtaccctgagcagtgacatcagtgtcggccactctgctgttactggagccggcagaagccagcgagccctcctcggtcctccggtcctaccgctcagactccagtaaggaccaggctccagggtccccgtgggttttctggatccaaagatacctcggccaacgtgggcctcctgctcatctctgggctgcagcctgagcatgaagctgactctgaccatgcaggctggtgcaacagggcttct

SEQ ID NO: 166 - DNA, 245 bp, Bos taurus
tgcaccccgagcagtgacatcagtgttggctgctctgctgttactggaaccagcagaagccagcgagccctccttagtcctccagtcctaccactcagactccagtaagaaccagtctttggggtccccgcgggttttctggatccaaagatgcctcagccaacgcggggctcctgctcgtctctgggctgcagcctgaggatgaggctatctctaaccatgcaggctggtgcaacagggcttct

SEQ ID NO: 167 - DNA, 245 bp, Bos taurus
tgcaccctgagcagtgacatcaatgttggctgctctgctgttactggaaccagcagaagccagcgagccctccttagtcctccggtcctaccactcagactccagtaagaaccagtctttggggtccccgcgggttttctggatccaaagatgcctcagccaacgcggggctcctgctcgtctctgggctgcagcctgaggatgaggctatctctaaccatgcaggctggtgcaacagggcttct

SEQ ID NO: 168 - DNA, 245 bp, Bos taurus
tgcaccctgagcagtgacatcagtgtcggccgctctgctgttactggaaccagcagaagccagcgagccctcctcggtcctccggtcctaccactcagattccagtaagaaccaggctccggggtccccatgggttttctggatccaaagatgcctcggccaatgcggggctcctgctcgtctctgggctacagcttgaggatgaggctgactctgaccatgcaggctggtgcaacagggctcct

SEQ ID NO: 169 - DNA, 246 bp, Bos taurus
tgcacccggagcagtgacatcagtgtcggccgctctgctgttactagaaccagcagaagccagtgagccctccttggtcctccagttctaccactcagactccagtatgaaccgggctccaggatcccccgcgggttttctggatccaaagatgcctcagccaacgcagggctccttcttgtctctgggctgcagcctgagcacgaggctgactctgaccgtgcaggctggtgcaacagggcttct

SEQ ID NO: 170 - DNA, 246 bp, Bos taurus
tgcaccctgcgcagtgacatcagtgtcggccactctgctcttactggaaccagcagaagccagcgagccctcctcggtcctctggtcctaccactgagactccagtaagaatcaggctccggggtcccccgtgggttttctggatccaaagatgcctcggccaatgtagggctcctgctcttctctgggctgcagcccgaggacgaggctgactctgaccgtgcaggctggtgcaacagggcttct

SEQ ID NO: 171 - DNA, 245 bp, Bos taurus; identical to SEQ ID NO: 167

SEQ ID NO: 172 - DNA, 245 bp, Bos taurus
tgcaccccgagcagtgacatcagtgtcagtcgctctgctgttactagaaccagcagaagccagcgagccctccttagtcctccggtcctaccactcagaccccagtaagaaccagtctttggggtccccgcgggttttctggatccaaagatgcctcagccaacgcggggctcctgctcgtctctgggctgcagcctgaggatgaggctgactctgaccatgcaggctggtgcaacagggcttct

SEQ ID NO: 173 - DNA, 206 bp, Bos taurus
gttactggaaccagcagaagccagtgagccctcctccgccctccgatcctaccactcagactccagtaagaaccaggctccggggtcctcgcaggttttctggatccaaagatgcctcggccaatgcagggctcctgctcgtctccgggctgcagcctgaggatgaggctgactctgaccgtgcaggctggtgcaacagggcttct

SEQ ID NO: 174 - DNA, 198 bp, Bos taurus
tgttactggaaccagcagaagccagcgagccctccttagtcctccggtcctaccactcagactccagtaagaaccagtcggggtccccgcgggttttctggatccaaagatgcctcagccaaggggctcctgctcgtctctgggctgcagcctgaggatgaggctactctaaccatgcaggctggtgcaacagggctt

SEQ ID NO: 175 - DNA, 206 bp, Bos taurus
gttactggaaccagcagaagccagtgagcctcctccgccctccgatcctaccactcagactccagtacagaaccaggctccggggtcctcgcaggttttctggatccaaagatgcctcggccaatgcagggctcctgctcgtctccgggctgccacctgaggataggctggactctgaccgtgcaggctggtgcaacagggcttct

SEQ ID NO: 176 - DNA, 38 bp, Bos taurus
ttttgtcttaggcggcgggacctgggtcaccgtcctgg

SEQ ID NO: 177 - DNA, 38 bp, Bos taurus
tgatcttttcggcggcgggaccagagtgaccgtcctgg

SEQ ID NO: 178 - DNA, 38 bp, Bos taurus
tgatcttttcggcggcgggaccacagtgaccgtcctgg

SEQ ID NO: 179 - DNA, 38 bp, Bos taurus
tgctgttttcggcagcgggaccacactgaccgtcctgg

SEQ ID NO: 180 - DNA, 38 bp, Bos taurus
tcctattttcattggcaggaccaggctgactgtcctgg

SEQ ID NO: 181 - DNA, 38 bp, Bos taurus; identical to SEQ ID NO: 179

SEQ ID NO: 182 - DNA, 38 bp, Bos taurus; identical to SEQ ID NO: 179

SEQ ID NO: 183 - DNA, 38 bp, Bos taurus; identical to SEQ ID NO: 180

SEQ ID NO: 184 - DNA, 306 bp, Bos taurus
  modified_base (1)..(1): a, c, t, g, unknown or other
nagagtgaaaccagccccagcatcttcccgctgagccttgggaacaacgacccagccgggcaggtggtcatcggctgcctggtccagggcttcttcccgtcggcacccctgagcgtgacctggaaccagaatggcgacagcgtgtccgtcaggaacttccctgccgtgctggccgggagcctgtacaccatgagcagccagctgaccttgccggccagcctgtgcccaaaaggccagtccgtgacctgccaagtgcagcacctctccaaagccagcaagaccgtggccgtgccctgcataattcaa

SEQ ID NO: 185 - DNA, 330 bp, Bos taurus
gactcaagttcatgttgcgtgccgaactgcgagcccagcctgtccgtgcagccaccagccctcgaggacctgctcctgggctccaacgccagcctcacgtgcacactgagtggcctgaaaagcgccgagggcgccagcttcacctggaacccgacaggtgggaagaccgccgtccaggggtcgcccaagcgtgactcctgtggctgctacagcgtgtccagcgtcctgccgggctgtgccgatccctggaacagtggacagactttctcctgctctgtcacccaccccgagtccaagagttcactgaccgccaccatcaagaaagactta

SEQ ID NO: 186 - DNA, 393 bp, Bos taurus
gggaacacgttccggcctcaggtccacctgctgccgccgccgtcggaggagctggccctcaacgagctggtgacgctgacgtgcctggtgcggggattcagccccaaggaggtgctggtgcgttggctgcagggcaatcaagagctgccccgcgagaagtatctgacctggggccccctgcccgaggctggccagagcgtcaccaccttcgccgtgaccagcgtgctacgcgtggacgccgaggtctggaagcagggggacaccttctcctgcatggtgggccacgaggccctgcccctggccttcacccagaagaccatcgaccgcctggcgggtaaacccacccacgtgaacgtgtccgtggtcatgtcagaggtggatggggtctgctac

SEQ ID NO: 187 - DNA, 186 bp, Bos taurus
gaacatcagccctggctggtgctggacctgatgcagagcagccccgaggaggacagcccagaggccagcctgtggcccacgaccgtcaccctgctcaccctcttcctgctgagcctcttctacagcacagcactgactgtgacgagcatccggaccacgccggacagccgggaggtcccccagtac

SEQ ID NO: 188 - DNA, 324 bp, Bos taurus
aaggtgaatcacacctgagagtcttccccctggtgtcctgcgtgagctccccatccgatgagagcacggtggccctgggctgcctggcccgggacttcgtgcccaattcagtcagcttctcctggaagttcaacaacagcacagtcagcagcgagagattctggaccttccccgaagtcctgagggacggcttgtggtcggcctcctctcaggtggtcctgccctcctcaagcgcctttcaagggccggatgactacctggtgtgtgaagtccagcaccccaagggaggaaagaccgtcggaaccgtgagggtggtccccagag

SEQ ID NO: 189 - DNA, 90 bp, Bos taurus
catcgactccaaccccgaccactccattgccttctctgatatccgggtcagagggctccaacaaggcggtcagcacgcagagcagcccag

SEQ ID NO: 190 - DNA, 66 bp, Bos taurus
cactgaccaccagccacagacagacagaagcccagacactggcgtgtccaaaggaaccctgcagag

SEQ ID NO: 191 - DNA, 324 bp, Bos taurus
agtgtcagaaccacacccaggcccccagagtccacctgctgcccccaaccccccagggcctttggctcctggacaaggccgagttcacctgcctggccacgggggaggccccgctggatgcccacttctcctgggaggtgtacgggcagccccacggcggggccttggaggagggacccaccaggcacataaacagctcctggagccagagcagccgcctggccctgcccaggtccctgtgggcctcgggctccaacgtcacctgcacactgagcagccctggcctgcagtcgccggtgaccctgacggctcagagagaacatg

SEQ ID NO: 192 - DNA, 321 bp, Bos taurus
ccgcctcagtgcctggcaatctgaccctccgcactgtgaccgcgcctggccccttctcccctgcctggctcctgtgcgaggtgtccggcttctcacccgtggacatcctcctcacgtggctggagagccagcaagaagtggagccttcccagtttgccacggcgcacaccacggcccaggctgggcgtgcctcatcccacacctggagtgtcctgcgtgtctccagccccctggaccacgcgggggccacctacacctgtgtggtcagccacgaggcctcccggacgctcctcaatggcagctgcagcctggacactggtg

SEQ ID NO: 193 - DNA, 147 bp, Bos taurus
gtctggccacctggccaccggtggagcccaggacgagaagcagcgattgacggcacggatgtggaggatgccagcccactctggctcaccttcctggccctcttcctcgtcactgtggtctacggcggcttcgtcaccttcatcaag

SEQ ID NO: 194 - DNA, 6 bp, Bos taurus
gtgaag

SEQ ID NO: 195 - DNA, 324 bp, Bos taurus
aaggtgaatcgctcccgagagtcttccccttggtgtcctgcatgagctccccgtctgatgagagaatggtggccctgggctgcctggcccggatcttcatacccaattcgttcagcttctcctggaagttaaacaacagcacagtcagcagcgagagattctggaccttccccgcagtcctgagggacggcttgtggtcggcctcctctcaggtggccctgtcctcctcgagcgcctttcaagggccggatgactacctggtgtgtgaagtccagcaccccaagggaggaaagaccctcggccccgtgagggtgggccccagag

SEQ ID NO: 196 - DNA, 185 bp, Bos taurus
ctcctgcctgtcattcacaggagctctcctgtgcgtctgagaagacctccctgacctccatggctgggccatggggcagctgggacccctggcctttacccgaacggagctcatccagggggtcctgtcatcgcatttagccgcctcaccggccccagaccactcacgcctgcattccatgtgtc

SEQ ID NO: 197 - DNA, 90 bp, Bos taurus; identical to SEQ ID NO: 189

SEQ ID NO: 198 - DNA, 66 bp, Bos taurus
cgccggccaccagccacagacagacagaagcccggacactggcatgtccaaaggacccctgcagag

SEQ ID NO: 199 - DNA, 325 bp, Bos taurus
agtgtcagaaccacacccaggcccccagcgtccacctactgcccccaaaacccgcagggcctctggctcctggacaaggccgagttcacctgcctggccatgggggaggccccaccggatgtccacttctcctgggaggtgaacgggcagccccacggcgcggccttggaggagggacccacctggcacatgaacggctcctggagccagagcagccgcctggccctgcccaggtccctgtgggcctcaggctccaacgtcacctgcacactgagtggccccggcctgcggtcgccggtgaccctgatggctcagagagaacatg

SEQ ID NO: 200 - DNA, 321 bp, Bos taurus
ccgcctcagtgcctggcaatctgaccctccgcactgtgaccgcgcctggccccttctcccctgcctggctcctgtgcgaggtgtccggcttctcacccgtggacatcctcctcacgtggctggagggccagcaagaagtggagccttcccagtttgccacggcacacaccacagcccaggctgggcacgcctcatcccacacctggagtgtcctgcgtgtctccagccccctggaccacgtgggggccacctacacctgtgtggtcagccacgaggcctcccggacgctcctcaatggcagctgcagcctggacactggtg

SEQ ID NO: 201 - DNA, 143 bp, Bos taurus
gtctggccacctggccgccctggagccaggatgagagcagcgacgacggcacggatgtggaggatgccagcccactctggctcaccttcctggccctcgtcctcatcactgtggtctacggcggctttgtcaccttcatcaag

SEQ ID NO: 202 - DNA, 6 bp, Bos taurus
gtgaag

SEQ ID NO: 203 - DNA, 100 bp, Bos taurus
ttctcaagcacctttcaagggccggatgactacctggtgtgcgaagtccagcaccccaagggaggaaagaccgttggaaccgtgagggtggtccccagag

SEQ ID NO: 204 - DNA, 184 bp, Bos taurus
ctcctgcctgtcattcacacgagctctcctgtgcgtctgagaagacctccctgactccatggctgggccatggggcagccgggacccctggcctttacccgaacggagctcatccagggggtcctgtcatcgcatttagccgcctcaccggccccagaccactcacccctgcattccatgtgtc

SEQ ID NO: 205 - DNA, 90 bp, Bos taurus
catcgactccaaccccgaccacttcagtgccttctctgatatccgggtcagagggctccatcaaggccgtcagcacgcagagcagcccag

SEQ ID NO: 206 - DNA, 324 bp, Bos taurus
agtgtcagaaccacacccaggcccccagcgtccacctgctgcccccaaccccccagggcctctggctcctggacaaggccgagttcacctgcctggccacgggggaggccccgctggatgcccgcttctcctgggaggtgaatgggcagccccacggcggggccttggaggagggacccacctggcacatgaacagctcctggagccagagcagccgcctggccctgcccaggtccctgtgggcctcaggctccaacgtcacctgcacactgagtggcccctgcctgcggtcaccggtgaccctgatggctcagagagaacatg

SEQ ID NO: 207 - DNA, 321 bp, Bos taurus
ccgcctcagtgcccggcaatctgaccctccgcactgtgaccgcgcctggccccttctcccatgcctggctcctgtgcaaggtttccggcttctcacccgtggacatcctcctcacgtggctggagagccagcaagaagtggagccttcccagtttgccacggcgcacaccacggcccaggctgggcatgcctcatcccacacctggagtgtcctgcgtgtctccagccccctggaccacgcgggggccacctacacctgtgtggtcagccacgaggcctcccggacgctcctcaatggcagctgcagcctggacactggtg

SEQ ID NO: 208 - DNA, 143 bp, Bos taurus
gtctggccacctggccaccgtggagccaggacgagagcagcgacgacggcacggatgtggaggatgccagcccactctggctcaccttcctggccctcttcctcgtcactgtggtctacggcggcttcgtcaccttcatcaag

SEQ ID NO: 209 - DNA, 6 bp, Bos taurus
gtgaag

SEQ ID NO: 210 - DNA, 100 bp, Bos taurus; identical to SEQ ID NO: 203

SEQ ID NO: 211 - DNA, 184 bp, Bos taurus; identical to SEQ ID NO: 204

SEQ ID NO: 212 - DNA, 90 bp, Bos taurus; identical to SEQ ID NO: 205

SEQ ID NO: 213 - DNA, 324 bp, Bos taurus
agtgtcagaaccacacccaggcccccagcgtccacctgctgcccccaaccccccagggcctctggctcctggacaaggccgagttcacctgcctggccacgggggaggccccgctggatgcccgcttctcctgggaggtaaatgggcagccccacggcggggccttggaggagggacccacctggcacatgaacagctcctggagccagagcagccgcctggccctgcccaggtccctgtgggcctcaggctccaacgtcacctgcacactgagtggcccctgcctgcggtcaccggtgaccctgatggctcagagagaacatg

SEQ ID NO: 214 - DNA, 321 bp, Bos taurus
ccgcctcagtgcccggcaatctgaccctccgcactgtgaccgtgcctggccccttctcccatgcctggctcctgtgcgaggtgtccggcttctcacccgtggacatcctcctcacgtggctggagagccagcaagaagtggagccttcccagtttgccacggcgcacaccacggcccaggctgggcgtgcctcatcccacacctggagtgtcctgcgtgtctccagccccctggaccacgcgggggccacctacacctgtgtggtcagccacgaggcctcccggacgctcctcaatggcagctgcagcctggacactggtg

SEQ ID NO: 215 - DNA, 143 bp, Bos taurus; identical to SEQ ID NO: 208

SEQ ID NO: 216 - DNA, 6 bp, Bos taurus
gtgaag

SEQ ID NO: 217 - DNA, 291 bp, Bos taurus
  modified_base (1)..(1): a, c, t, g, unknown or other
ncctccatccaggctccatccatctaccccttgaggctctgttgcacagaagaagcccgtgtaaggctgggctgcctggtcaaggactacttgccagggtcagtgactgtgacctgggacacagtgcccctggatggaagcaccctgaccttccctagcatccaaatggcgagctccagtctctacattaccaccagccagctgaccatctcgggcgagcagcccaaggagttcacctgcagagttttacacgctgagaccaactccaacttgaataagaccatcagcact

SEQ ID NO: 218 - DNA, 324 bp, Bos taurus
gagtgcgccaagaacttcagcgacccctcagtgaagctcttctactcctcctgcaaccccaatggcgacacccagaccaccatccacctcctgtgccggatctccggctacaccccgggcaaaatcaaggtcacctggctggtggatgggctcaagtccgaagagctgtatgcacgatccggccctgagatacaggagggcaatctgacctccacctacagtgaagtcaacatcacacagggccagtgggtgtccgagaaaacctacacctgccgggtcaactattacggctacaacttcgaaagccacgcccacaggtgcaca

SEQ ID NO: 219 - DNA, 324 bp, Bos taurus
gccgagtccgagccccgcggcgtgagcgcctacctgagcccacccacccccctcgagctgtacgtcaacaagtcacccaagatcacctgcctggttgtggacctggccaacgagaagaacttgagcctgacctggtcgagggcaaacgggaagcctgtgcacgcaggcccccctgagatcaagcgtcagttcaacgggacggtcaccgtcacgtccaccctgccggtggacgtcactgactgggtagaaggcgagacctactactgcaaagtgagccacagcgacctgcccacggacatccagcgatccatctccaaggatgtt

SEQ ID NO: 220 - DNA, 339 bp, Bos taurus
ggcaagcgtctggcccccaaggcctacgtgttcttgccagacggaaaggagctggagaacgaggaggagctcaccctcacctgcatgatccagaaattcttccccagggacatctttgtgcggtggctgcataacaaggaactgatgcgggcagaccagcacaccaccacacagccccacagggccgacaacaacaccccagccttcttcgcctacagccgcctggcggtccctagggccaactggaagaggggcgatgagttcacctgccaagtgatccatgaggcactgcccaggactaggaccctggagaaatcggtgttcattaacagcggtaaa

SEQ ID NO: 221 - DNA, 135 bp, Bos taurus
gagctggccctcgaggacctgtgtgcagaggaagctgagagcgaggagctggaggagacctggaccagcctccttgtcttcatcgtgctcttcctgctcagcatgagctatggcgccgccgtcagcctctgcaag

SEQ ID NO: 222 - DNA, 93 bp, Bos taurus
gtgaagtggatcctggccgccatcctccaggggcagccccagggctcccaagactacaccaacgtcacacagcgcccactgcctgctggtgtc

SEQ ID NO: 223 - DNA, 291 bp, Bos taurus
  modified_base (1)..(1): a, c, t, g, unknown or other
ncctccaccacagccccgaaagtctaccctctgagttcttgctgcggggacaagtccagctccaccgtgaccctgggctgcctggtctccagctacatgcccgagccggtgaccgtgacctggaactcgggtgccctgaagagcggcgtgcacaccttcccggctgtccttcagtcctccgggctctactctctcagcagcatggtgaccgtgcccggcagcagctcaggacagaccttcacctgcaacgtagcccacccggccagcagcaccaaggtggacaaggctgtt

SEQ ID NO: 224 - DNA, 36 bp, Bos taurus
gatcccagatgcaaaacaacctgtgactgttgccca

SEQ ID NO: 225 - DNA, 330 bp, Bos taurus
ccgcctgagctccctggaggaccctctgtcttcatcttcccaccgaaacccaaggacaccctcacaatctcgggaacgcccgaggtcacgtgtgtggtggtggacgtgggccacgatgaccccgaggtgaagttctcctggttcgtggacgacgtggaggtaaacacagccacgacgaagccgagagaggagcagttcaacagcacctaccgcgtggtcagcgccctgcgcatccagcaccaggactggactggaggaaaggagttcaagtgcaaggtccacaacgaaggcctcccggcccccatcgtgaggaccatctccaggaccaaa

SEQ ID NO: 226 - DNA, 327 bp, Bos taurus
gggccggcccgggagccgcaggtgtatgtcctggccccaccccaggaagagctcagcaaaagcacggtcagcctcacctgcatggtcaccagcttctacccagactacatcgccgtggagtggcagagaaatgggcagcctgagtcagaggacaagtacggcacgacccctccccagctggacgccgacggctcctacttcctgtacagcaggctcagggtggacaggaacagctggcaggaaggagacacctacacgtgtgtggtgatgcacgaggccctgcacaatcactacacgcagaagtccacctctaagtctgcgggtaaa

SEQ ID NO: 227 - DNA, 135 bp, Bos taurus
gacctgctgctggaggaggagatctgtgcggacgcccaggacggggagctggacgggctctggacgactatctccatcttcatcacactcttcctgctcagcgtctgctacagcgccaccgtgaccctcttcaag

SEQ ID NO: 228 - DNA, 81 bp, Bos taurus
gtgaagtggatcttctcatcagtggtggagctgaagaggacgatcgtccccgactacagaaatatgatcgggcagggagcc

SEQ ID NO: 229 - DNA, 291 bp, Bos taurus
  modified_base (1)..(1): a, c, t, g, unknown or other
ncctccaccacagccccgaaagtctaccctctggcatcccgctgcggagacacatccagctccaccgtgaccctgggctgcctggtctccagctacatgcccgagccggtgaccgtgacctggaactcgggtgccctgaagagcggcgtgcacaccttcccggccgtccttcagtcctccgggctctactctctcagcagcatggtgaccgtgcccggcagcagctcaggacagaccttcacctgcaacgtagcccacccggccagcagcaccaaggtggacaaggctgtt

SEQ ID NO: 230 - DNA, 39 bp, Bos taurus
ggggtctccattgactgctccaagtgtcataaccagcct

SEQ ID NO: 231 - DNA, 321 bp, Bos taurus
tgcgtgagggaaccatctgtcttcatcttcccaccgaaacccaaagacaccctgatgatcacaggaacgcccgaggtcacgtgtgtggtggtgaacgtgggccacgataaccccgaggtgcagttctcctggttcgtggatgacgtggaggtgcacacggccaggtcgaagccaagagaggagcagttcaacagcacgtaccgcgtggtcagcgccctgcccatccagcaccaggactggactggaggaaaggagttcaagtgcaaggtcaacaacaaaggcctctcggcccccatcgtgaggatcatctccaggagcaaa

SEQ ID NO: 232 - DNA, 327 bp, Bos taurus
gggccggcccgggagccgcaggtgtatgtcctggacccacccaaggaagagctcagcaaaagcacgctcagcgtcacctgcatggtcaccggcttctacccagaagatgtagccgtggagtggcagagaaaccggcagactgagtcggaggacaagtaccgcacgaccccgccccagctggacaccgaccgctcctacttcctgtacagcaagctcagggtggacaggaacagctggcaggaaggagacacctacacgtgtgtggtgatgcacgaggccctgcacaatcactacatgcagaagtccacctctaagtctgcgggtaaa

SEQ ID NO: 233 - DNA, 135 bp, Bos taurus
gacctgctgctggaggaggagatctgtgcggacgcccaggacggggagctggacgggctctggacgactatctccatcttcatcacactctttctgctcagcgtctgctacagcgccaccgtgaccctcttcaag

SEQ ID NO: 234 - DNA, 81 bp, Bos taurus
gtgaagtggatcctctcatccgtggtggagctgaagcagtcgatcactcccaactacagaaacatgatcggacagggcgcc

SEQ ID NO: 235 - DNA, 294 bp, Bos taurus
  modified_base (1)..(1): a, c, t, g, unknown or other
ncctccaccacagccccgaaagtctaccctctggcatccagctgcggagacacatccagctccaccgtgaccctgggctgcctggtctccagctacatgcccgagccggtgaccgtgacctggaactcgggtgccctgaagagcggcgtgcacaccttcccggccgtccggcagtcctctgggctgtactctctcagcagcatggtgaccgtgcccgccagcacctcaggaacccagaccttcacctgcaacgtagcccacccggccagcagcaccaaggtggacaaggctgtc

SEQ ID NO: 236 - DNA, 66 bp, Bos taurus
actgcaaggcgtccagtcccgacgacgccaaagacaaccatccctcctggaaaacccacaacccag

SEQ ID NO: 237 - DNA, 45 bp, Bos taurus
gagcctgaagttgaaaagacaccctgccagtgttccaaatgccca

SEQ ID NO: 238 - DNA, 324 bp, Bos taurus
gaacctccgggaggactgtctgtcttcatcttcccaccgaaacccaaggacaccctcacaatctcaggaacgcccgaggtcacgtgtgtggtggtggacgtgggccaggatgaccccgaggtgcagttctcctggttcgtggacgacgtggaggtgcacacggccaggacgaagccgagagaggagcagttcaacagcacctaccgcgtggtcagcgccctgcgcatccagcaccaggactggctgcagggaaaggagttcaagtgcaaggtcaacaacaaaggcctcccggcccccattgtgaggaccatctccaggaccaaa

SEQ ID NO: 239 - DNA, 327 bp, Bos taurus
gggcaggcccgggagccgctggtgtatgtcctggccccaccccgggaagagctcagcaaaagcacgctcagcctcacctgcctgatcaccggtttctacccagaagagatagacgtggagtggcagagaaatgggcagcctgagtcagaggacaagtaccacacgaccgcaccccagctggatgctgacggctcctacttcctgtacagcaggctcagggtgaacaagagcagctggcaggaaggagaccactacacgtgtgcagtgatgcatgaagctttacggaatcactacaaagagaagtccatctcgaggtctccgggtaaa

SEQ ID NO: 240 - DNA, 135 bp, Bos taurus
gacttgctgctggaggaggagatctgtgcggacgacctggatggggagctggacgggctctggacgactatctccatcttcatcacactcttcctgctcagcgtctgctacagcgccactgtgaccctcttcaag

SEQ ID NO: 241 - DNA, 81 bp, Bos taurus
gtgaaatggatcttctcctcggcggtggagctgaagaggacgatcgtccccgactacagaaacatgctcgggcagggcgcc

SEQ ID NO: 242 - DNA, 294 bp, Bos taurus; identical to SEQ ID NO: 235
  modified_base (1)..(1): a, c, t, g, unknown or other

SEQ ID NO: 243 - DNA, 66 bp, Bos taurus; identical to SEQ ID NO: 236

SEQ ID NO: 244 - DNA, 45 bp, Bos taurus; identical to SEQ ID NO: 237

SEQ ID NO: 245 - DNA, 324 bp, Bos taurus; identical to SEQ ID NO: 238

SEQ ID NO: 246 - DNA, 327 bp, Bos taurus; identical to SEQ ID NO: 239

SEQ ID NO: 247 - DNA, 135 bp, Bos taurus; identical to SEQ ID NO: 240

SEQ ID NO: 248 - DNA, 81 bp, Bos taurus; identical to SEQ ID NO: 241

SEQ ID NO: 249 - DNA, 288 bp, Bos taurus
cctccaccacagccccgaaagtctaccctctggcatccagctgcggagacacatccagctccaccgtgaccctgggctgcctggtctccagctacatgcccgagccggtgaccgtgacctggaactcgggtgccctgaagagcggcgtgcacaccttcccggccgtccggcagtcctctgggctgtactctctcagcagcatggtgaccgtgcccgccagcagctcagaaacccagaccttcacctgcaacgtagcccacccggccagcagcaccaaggtggacaagg

SEQ ID NO: 250 - DNA, 45 bp, Bos taurus
agtctgaagttgaaaagacaccctgccagtgttccaaatgcccag

SEQ ID NO: 251 - DNA, 324 bp, Bos taurus
aacctctgggaggactgtctgtcttcatcttcccaccgaaacccaaggacaacctacacatctcgggaacgcccgaggttacgtgtgtggtggtggacgtgggccaggatgaccccgaggtgcagttctcctggttcgtggacgacgtggaggtgcacacggccaggacgaagccgagagaggagcagttcaacagcacctaccgcgtggtcagcgccctgcgcatccagcaccaggactggctgcagggaaaggagttcaagtgcaaggtcaacaacaaaggcctcccggcccccattgtgaggaccatctccaggaccaaag

SEQ ID NO: 252 - DNA, 325 bp, Bos taurus
ggcaggcccgggagccgcaggtgtatgtcctggccccacccgggaagagctcagcaaaagcacgctcagcctcacctgcctgatcaccggtttctacccagaagagatagacgtggagtggcagagaaatgggcagcctgagtcggaggacaagtaccacacgaccgcaccccagctggatgctgacggctcctacttcctgtacagcaggctcagggtgaacaagagcagctggcaggaaggagaccactacacgtgtgcagtgatgcatgaagctttacggaatcactacaaagagaagtccatctcgaggtctccgggtaaa

SEQ ID NO: 253 - DNA, 324 bp, Bos taurus
  modified_base (1)..(1): a, c, t, g, unknown or other
naaggtgaatcacacccgaaagtcttccccctggtgtcctgcgtgagctcgccatccgatgagagcacggtggccctgggctgcctggcccgggacttcgtgcccaattcagtcagcttctcctggaagttcaacaacagcacagtcagcagcgagagattctggaccttccccgaagtcctgagggacggcttgtggtcggcctcctctcaggtggtcctgccctcctcaagcgcctttcaagggccggatgactacctggtgtgcgaagtccagcaccccaagggaggaaagaccgtcggcaccgtgagggtgatcgctaca

SEQ ID NO: 254 - DNA, 333 bp, Bos taurus
aaggcggaagtgctgtccccagtcgtgagtgtctttgtcccgcctcgcaacagcctctctggtgacggcaatagcaagtccagcctcatctgccaggccacggacttcagccccaaacagatctcgttgtcctggtttcgtgatggaaagcggatagtgtctggaatttctgaaggccaggtggagactgtgcagtcctcacccataaccttcagggcctacagcatgctgaccatcacggagagagactggctcagccagaacgcgtacacctgccaggtagaacacaacaaggaaaccttccagaagaacgtgtcctcctcatgtgatgtt

SEQ ID NO: 255 - DNA, 315 bp, Bos taurus
gcaccaccatctccgatcggggtcttcaccatccccccatccttcgccgacatcttcctcacgaagtcagccaagctgtcctgtctggtcacaaacctggcctcctatgatggcctgaacatcagctggtcccgtcagaacgccaaggccctggagacccacacgtattttgagcgacacctcaacgacaccttcagcgcccggggtgaggcctcggtctgctcggaggactgggagtccggagaggagttcacgtgcacagtggcccactcggacctgcccttcccagaaaagaacgccgtctccaagcccaaa

SEQ ID NO: 256 - DNA, 393 bp, Bos taurus
gacgtcgccatgaaaccgccgtccgtgtacctgctgcctccaacgcgggaacagctgagcctgcgcgagtcggcctccgtcacctgcctggtgaaggcgttcgcgcccgcggacgtgttcgtgcagtggctgcagaggggggagcccgtgaccaagagcaagtacgtgaccagcgcccgcgcgcccgagccccaggaccccagcgtggtgtactttgtgcacagcatcctgacggtggccgaggaggactggagcaaaggggagacctacacctgcgtcgtgcacgaagccctgccccacatggtcaccgagcggaccgtggacaagtccaccggtaaacccaccctgtacaacgtgtccctggtcctgtctgacacagccagcacctgctac

SEQ ID NO: 257 - DNA, 117 bp, Bos taurus
gagggggaggtgagcgccgaggaagaaggctttgaaaacctcaacaccatggcctccaccttcatcgtgctcttcctcctgagcctcttctacagcaccacggtcaccctgttcaag

SEQ ID NO: 258 - DNA, 6 bp, Bos taurus
gtgaag

SEQ ID NO: 259 - DNA, 324 bp, Bos taurus
  modified_base (1)..(1): a, c, t, g, unknown or other
naaggtgaatcacacccgagagtcttccccctggtgtcctgcgtgagctccccatccgatgagagcacggtggccctgggctgcctggcccgggacttcgtgcccaattcagtcagcttctcctggaagttcaacaacagcacagtcagcagcgagagattctggaccttccccgaagtcctgagggacggcttgtggtcggcctcctctcaggtggtcctgccctcctcaagcgcctttcaagggccggatgactacctggtgtgcgaagtccagcaccccaagggaggaaagaccgtcggcaccgtgagggtggtcgctaca

SEQ ID NO: 260 - DNA, 333 bp, Bos taurus
aaggcggaagtgctgtccccagtcgtgagtgtctttgtcccgcctcgcaacagcctctctggtgacggcaatagcaagtccagcctcatctgccaggccacggacttcagccccaaacagatctccttgtcctggtttcgtgatggaaagcggatagtgtctggcatttctgaaggccaggtggagactgtgcagtcctcacccgtaactttcagggcctacagcatgctgaccatcacggagagagactggctcagccagaacgtgtacacctgccaggtagaacacaacaaggaaaccttccagaagaacgtgtcctcctcatgtgatgtt

SEQ ID NO: 261 - DNA, 315 bp, Bos taurus
gcaccaccatctcccatcggggtcttcaccatccccccatccttcgccgacatcttcctcacgaagtcagccaagctgtcctgtctggtcacaaacctggcctcctatgatggcctgaacatcagctggtcccgtcagaacggcaaggccctggagacccacacgtattttgagcgacacctcaacgacaccttcagcgcccggggtgaggcctcggtctgctcggaggactgggagtccggagaggagttcacgtgcacagtggcccactcggacctgcccttcccagaaaagaacaccgtctccaagcccaaa

SEQ ID NO: 262 - DNA, 393 bp, Bos taurus
gatgtcgccatgaaaccgccgtccgtgtacctgctgcctccaacgcgggaacagctgagcctgcgggagtcggcctccgtcacctgcctggtgaagggcttcgcgcccgcggacgtgttcgtgcagtggctgcagaggggggagcccgtgaccaagagcaagtacgtgaccagcagcccggcgcccgagccccaggaccccagcgtgtactttgtgcacagcatcctgacggtggccgaggaggactggagcaaaggggagacctacacctgcgtcgtgggccacgaggccctgccccacatggtcaccgagcggaccgtggacaagtccaccggtaaacccaccctgtacaacgtgtccctggtcctgtctgacacagccagcacctgctac

SEQ ID NO: 263 - DNA, 117 bp, Bos taurus
gagggggaggtgagcgccgaggaggaaggctttgagaacctcaacaccatggcctccaccttcatcgtgctcttcctcctgagcctcttctacagcaccacggtcaccctgttcaag

SEQ ID NO: 264 - DNA, 6 bp, Bos taurus
gtgaag

SEQ ID NO: 265 - DNA, 324 bp, Bos taurus
  modified_base (1)..(1): a, c, t, g, unknown or other
nggtctgatgctgagccatccgtcttcctcttcaaaccatctgatgagcagctgaagaccggaactgtctctgtcgtgtgcttggtgaatgatttctaccccaaagatatcaatgtcaagtggaaagtggatggggttactcagagcagcagcaacttccaaaacagtttcacagaccaggacagcaagaaaagcacctacagcctcagcagcatcctgacactgcccagctcagagtaccaaagccatgacgcctatacgtgtgaggtcagccacaagagcctgactaccaccctcgtcaagagcttcagtaagaacgagtgt

SEQ ID NO: 266 - DNA, 316 bp, Bos taurus
gtcagcccaagtccgcaccctcggtcaccctgttcccgccccccaccgaggagctcagcgccaacaaggccaccctggtgtgtctcatcagtgacttctacccgggtagcgtgaccgtggcctggaaggcagacggcagcaccatcacccgcaacgtggagaccacccgggcctccaaacagagcaacagcaagtacgcggccagcagctactgagcctgacgggcagcgactggaaatcgaaaggcagttacagctgcgaggtcacgcacgaggggagcaccgtgacgaagacagtgaagacctcagcgtgttct

SEQ ID NO: 267 - DNA, 318 bp, Bos taurus
ggtcagcccaagtccccaccctcggtcaccctgttcccgccctccaaggaggagctcagcgccaacaaggccaccctggtgtgtctcatcagcgacttctacccgggtagcgtgaccgtggcctggaaggcagacggcagcaccatcacccgcaacgtgaagaccacccgggcctccaaacagagcaacagcaagtacgcggccagcagctacctgagcctgacagacagcgactggaaatcgaaaggcagttacagctgcgaggtcacgcacgaggggagcaccgtgacgaagacagtgaagacctcagcgtgttct

SEQ ID NO: 268 - DNA, 318 bp, Bos taurus
ggtcagcccaagtccccaccctcggtcaccctgttcccgccctccaaggaggagctcagcgccaacaaggccaccctggtgtgtctcatcagcgacttctacccgggtagcgtgaccgtggcctggaaggcagacggcagcaccatcacccgcaacgtggagaccacccgggcctccaaacagagcaacagcaagtacgcggccagcagctacctgagcctgacgagcagcgactggaaatcgaaaggcagttacagctgcgaggtcacgcacgaggggagcaccgtgacgaagacagtgaagacctcagcgtgttct

SEQ ID NO: 269 - DNA, 318 bp, Bos taurus
ggtcagcccaagtccccaccctcggtcaccctgttcccgccctccacggaggagctcaacggcaacaaggccaccctggtgtgtctcatcagcgacttctacccgggtagcgtgaccgtggtctggaaggcagacggcagcaccatcacccgcaacgtggagaccacccgggcctccaaacagagcaacagcaagtacgcggccagcagctacctgagcctgacgagcagcgactggaaatcgaaaggcagttacagctgcgaggtcacgcacgaggggagcaccgtgacgaagacagtgaagccctcagagtgttct

SEQ ID NO: 270 - DNA, 315 bp, Bos taurus
gtcagcccaagtccacacctcggtcaccctgttcccgccctccaaggaggagctcagcaccaacaaggccaccctggtgtgtctcatcagcgacttctacccgggtagcgtgaccgtggtctagaaggcagacggcagcaccatcacccacaacgtggagaccacccgggcctccaaacagagcaacagcaagtaccgcggccagcagctacctgagcctgatgggcagcgactggaaatcgaaaggcagttacagctgcgaggtcacgcacgagggagcaccgtgacgaagacagtgaagcctcagagtgttct

SEQ ID NO: 271 - DNA, 314 bp, Bos taurus
gtcagcccaagttcacaccctcgtcactgtttccgcccacctccaaggagagccagcaccaacaaggccaacccctgtgtgtctcatcagcgacttctaccccggtagtcgtacccgggtcagaaggcagaacggcaaccatctacccacaacgtggagaccacccggccccaaacagagcaccagcaagtaacgcggccgagcactacccacctgagcctgatggcagcgacggaaaatcgaaaggctagttacagcgcgagttcagcacgaaggggagcacgtgacgaaacatgaagcctcagagtgttcct

SEQ ID NO: 272 - DNA, 316 bp, Bos taurus
gtcagcccaagtccccaccctcgtcaccctgttcccgccctccacggaggagctcaacggcaacaaggccaccctggtgtgtctcatcagcgacttctacccgggtagcgtgaccgtggtctggaaggcagacggcagcaccatcacccgcaacgtggagaccacccgggcctccaaacagagcaacagcaagtacgcggccagcagctacctgagcctgacgagcagcgactggaaatcgaaaggcagttacagctgcgaggtcacgcacgaggggagcaccgtgacgaagacagtgaagccctcagagtgttct

SEQ ID NO: 273 - DNA, 318 bp, Bos taurus; identical to SEQ ID NO: 269

SEQ ID NO: 274 - DNA, 316 bp, Bos taurus
gtcagcccaagtccacaccctcggtcaccctgttcccgccctccaaggaggagctcagcaccaacaaggccaccctggtgtgtctcatcagcgacttctacccgggtagcgtgaccgtggtctagaaggcagacggcagcaccatcacccacaacgtggagaccacccgggcctccaaacagagcaacagcaagtacgcggccagcagctacctgagcctgatgggcagcgactggaaatcgaaaggcagttacagctgcgaggtcacgcacgaggggagcaccgtgacgaagacagtgaagcctcagagtgttct

SEQ ID NO: 275 - DNA, 24 bp, Artificial Sequence
  source: /note="Description of Artificial Sequence: Synthetic primer"
acataatacactgaaatggagccc

SEQ ID NO: 276 - DNA, 20 bp, Artificial Sequence
  source: /note="Description of Artificial Sequence: Synthetic primer"
gtccttggtcaacgtgaggg

SEQ ID NO: 277 - DNA, 24 bp, Artificial Sequence
  source: /note="Description of Artificial Sequence: Synthetic primer"
cataatacactgaaatggagccct

SEQ ID NO: 278 - DNA, 20 bp, Artificial Sequence
  source: /note="Description of Artificial Sequence: Synthetic primer"
gcaacagtggtaggtcgctt

SEQ ID NO: 279 - DNA, 100 bp, Mus musculus
atttctgtacctgatctatgtcaatatctgtaccatggctctagcagagatgaaatatgagacagtctgatgtcatgtggccatgcctggtccagacttg

SEQ ID NO: 280 - DNA, 100 bp, Mus musculus
gtcaatcagcagaaatccatcatacatgagacaaagttataatcaagaaatgttgcccataggaaacagaggatatctctagcactcagagactgagcac

SEQ ID NO: 281 - DNA, 1103 bp, Artificial Sequence
  source: /note="Description of Artificial Sequence: Synthetic polynucleotide"
gcattgaataaaccagtataaacaagcaagcaaagatagatagatagatagatagatagatagatagatacatagatagatagatagatagatagatgatagatagatagatagatagatagatttttacgtataatacaataaaaacattcattgtccctctattggtgactactcaaggaaaaaaatgttcatatgcaagaaaaaatgttatcattaccagatgatccagcaatctagcaatatatatattgtttattcacaaaacatgaatgaaccttttaagaagctgttacagtgtaaaaattaagttaaatcactgaagaacatatactgtgtgatttcattcaaatgaaatttgagaagtaaatatatatgtatatatatatatatgtaaaaaatataagtctgaactacaaaaattcaatttgtttgatatgtaagaataagaaaaattgacccccaaaatttgttaataattaggtatgtgtatttttatgaatatataagtataataatgcttatagtatacactattctgaatcacatttattccctaagtgtgttcccttgattataattaaaagtatattttttaaatacagagtcagagtacagtcaataaggcgaaaatatagttgaatgatttgcttcagcttttgtaatgtactagagattgtgagtacaaagtctcagagctcattttatccctgacaataaccagctctgtgcttcaagtacatttccatctttctctgaaatttagtcttatatagatagacaaaatttaagtaaatttcaaactacacagaacaactaagttgttgtttcatattgataatggatttgaactgcattaacagaactttaacatcctgcttattctcccttcagccatcatattttgctttattattttcactttttgagttatttttcacattcagaaagctcacataattgtcacttctttgtatactggtatacagaccagaacatttgcatattgttccctggggaggtctttgccctgttggcctgagataaaacctcaagtgtcctcttgcctccactgatcactctcctatgtttatttcctcaaa

SEQ ID NO: 282 - DNA, 49 bp, Artificial Sequence
  source: /note="Description of Artificial Sequence: Synthetic oligonucleotide"
atgagattctctgctcagctcctggggctcctcctgctctgggtcccag

SEQ ID NO: 283 - DNA, 401 bp, Artificial Sequence
  source: /note="Description of Artificial Sequence: Synthetic polynucleotide"
gtaagtacagagagggatgagaaggaggatgggggtgagttctggggcagcactgctctccacatgtgttctctgttagatgtgtatgacttgtcctgcagatgagcatgggaaccttagatcaatgatagtgaggaatgttccagaaggaagaaggtcctgtgctctggtcaggactgtgacaggggaagtggggatgatgtaggggatgtttagaggtctctttatacttcacagatatcaagttcattattgtgattgtacaattttgctgtatgatcacagacaatgtgagtaatacaaagtagtattaatgttttagctaaaataaatcagaaaatggaaacaataaaaatggttgctaatatttgtagctttctaattctctgtcattcctttag

SEQ ID NO: 284 - DNA, 308 bp, Artificial Sequence
  source: /note="Description of Artificial Sequence: Synthetic polynucleotide"
gatccagtggggatgttgtgctgacccagactccactctccctgtctatcatccctggagagatggcctccatctcctgcaagtctagtcagagcctggtacacagtgatggaaaaacctatttgaattggattcaatataaaccaggccaatcaccacagggtctgatctatcaggtttccaaccgttactctggggtctcagacaggttcactggcagtgggtcagggacagatttcacacttacaatcagcagagtgcaggctgaggatgctggagtctattactgttaccaaggtacagaagat

SEQ ID NO: 285 - DNA, 7 bp, Artificial Sequence
  source: /note="Description of Artificial Sequence: Synthetic oligonucleotide"
cacagtg

SEQ ID NO: 286 - DNA, 142 bp, Artificial Sequence
  source: /note="Description of Artificial Sequence: Synthetic polynucleotide"
atacagactctatcaaaaacttccttgcctggggcagcccagctgacaatgtgcaatctgaagaggagcagagagcatcttgtgtctgtgtgagaaggaggggctgggatacatgagtaattctttgcagctgtgagctctg

SEQ ID NO: 287 - DNA, 1103 bp, Artificial Sequence; identical to SEQ ID NO: 281
  source: /note="Description of Artificial Sequence: Synthetic polynucleotide"

SEQ ID NO: 288 - DNA, 49 bp, Artificial Sequence
  source: /note="Description of Artificial Sequence: Synthetic oligonucleotide"
atgatgagtcctgcccagttcctgtttctgttagtgctctggattcagg

SEQ ID NO: 289 - DNA, 386 bp, Artificial Sequence
  source: /note="Description of Artificial Sequence: Synthetic polynucleotide"
gtaaggagttttggaatgtgagggatgagaatggggatggagggtgatctctggatgcctatgtgtgctgtttatttgtggtggggcaggtcatatcttccagaatgtgaggttttgttacatcctaatgagatattccacatggaacagtatctgtactaagatcagtattctgacatagattggatggagtggtatagactccatctataatggatgatgtttagaaacttcaacacttgttttatgacaaagcatttgatatataatatttttaaatctgaaaaactgctaggatcttacttgaaaggaatagcataaaagatttcacaaaggttgctcaggatctttgcacatgattttccactattgtattgtaatttcag

SEQ ID NO: 290 - DNA, 11 bp, Artificial Sequence
  source: /note="Description of Artificial Sequence: Synthetic oligonucleotide"
aaaccaacggt

SEQ ID NO: 291 - DNA, 308 bp, Artificial Sequence; identical to SEQ ID NO: 284
  source: /note="Description of Artificial Sequence: Synthetic polynucleotide"

SEQ ID NO: 292 - DNA, 7 bp, Artificial Sequence
  source: /note="Description of Artificial Sequence: Synthetic oligonucleotide"
cacagtg

SEQ ID NO: 293 - DNA, 142 bp, Artificial Sequence; identical to SEQ ID NO: 286
  source: /note="Description of Artificial Sequence: Synthetic polynucleotide"

SEQ ID NO: 294 - DNA, 13 bp, Mus musculus
cttccttcctcag

SEQ ID NO: 295 - DNA, 13 bp, Artificial Sequence
  source: /note="Description of Artificial Sequence: Synthetic oligonucleotide"
aaattaattaacc